European Patent Application EP 4 729 636 A2, published April 22, 2026. Title: COMPOSITIONS AND METHODS FOR THE SELECTIVE DETECTION OF TUMOR-DERIVED VIRAL DNA. Applicant: The University of North Carolina at Chapel Hill. Application EP not yet assigned, filed March 16, 2021. The sequence listing filed with the application follows.

SEQUENCE LISTING (425 sequences)

SEQ ID NO: 1 - DNA, 19 bp, synthetic construct
  misc_feature 1..19: note = Synthetic Construct
  source 1..19: mol_type = other DNA
tgactctacgcttcggttg

SEQ ID NO: 2 - DNA, 19 bp, synthetic construct
  misc_feature 1..19: note = Synthetic Construct
  source 1..19: mol_type = other DNA
gcccattaacaggtcttcc

SEQ ID NO: 3 - DNA, 30 bp, synthetic construct
  misc_feature 1..30: note = Synthetic Construct
  source 1..30: mol_type = other DNA
cgtacaaagcacacacgtagacattcgtac

SEQ ID NO: 4 - DNA, 19 bp, synthetic construct
  misc_feature 1..19: note = Synthetic Construct
  source 1..19: mol_type = other DNA
ggtttgtaacatcccaggc

SEQ ID NO: 5 - DNA, 25 bp, synthetic construct
  misc_feature 1..25: note = Synthetic Construct
  source 1..25: mol_type = other DNA
gtgtattttttaaggggatcttctt

SEQ ID NO: 6 - DNA, 13 bp, synthetic construct
  misc_feature 1..13: note = Synthetic Construct
  misc_feature 6..7: note = locked nucleic acid
  misc_feature 9: note = locked nucleic acid
  source 1..13: mol_type = other DNA
cacctccagcacc

SEQ ID NO: 7 - DNA, 24 bp, synthetic construct
  misc_feature 1..24: note = Synthetic Construct
  source 1..24: mol_type = other DNA
atctgtacagcatgaagtgcaaga

SEQ ID NO: 8 - DNA, 19 bp, synthetic construct
  misc_feature 1..19: note = Synthetic Construct
  source 1..19: mol_type = other DNA
ctagtgggcgcatgtaggc

SEQ ID NO: 9 - DNA, 11 bp, synthetic construct
  misc_feature 1..11: note = Synthetic Construct
  misc_feature 2..4: note = locked nucleic acid
  misc_feature 5..7: note = locked nucleic acid
  source 1..11: mol_type = other DNA
tctatgacctg

SEQ ID NO: 10 - DNA, 20 bp, synthetic construct
  misc_feature 1..20: note = Synthetic Construct
  source 1..20: mol_type = other DNA
tgaagccagaattgagctag

SEQ ID NO: 11 - DNA, 18 bp, synthetic construct
  misc_feature 1..18: note = Synthetic Construct
  source 1..18: mol_type = other DNA
aggacagggtgttcagaa

SEQ ID NO: 12 - DNA, 13 bp, synthetic construct
  misc_feature 1..13: note = Synthetic Construct
  misc_feature 3: note = locked nucleic acid
  misc_feature 5..6: note = locked nucleic acid
  misc_feature 9: note = locked nucleic acid
  source 1..13: mol_type = other DNA
cagacgaccttcg

SEQ ID NO: 13 - DNA, 21 bp, synthetic construct
  misc_feature 1..21: note = Synthetic Construct
  source 1..21: mol_type = other DNA
agcacacaagtagatattcgc

SEQ ID NO: 14 - DNA, 19 bp, synthetic construct
  misc_feature 1..19: note = Synthetic Construct
  source 1..19: mol_type = other DNA
tagtagaacagttggggca

SEQ ID NO: 15 - DNA, 13 bp, synthetic construct
  misc_feature 1..13: note = Synthetic Construct
  misc_feature 4..5: note = locked nucleic acid
  misc_feature 7: note = locked nucleic acid
  misc_feature 9..10: note = locked nucleic acid
  misc_feature 13: note = locked nucleic acid
  source 1..13: mol_type = other DNA
taacagctcttgc

SEQ ID NO: 16 - DNA, 22 bp, synthetic construct
  misc_feature 1..22: note = Synthetic Construct
  source 1..22: mol_type = other DNA
taacaccacagttcgtttatgt

SEQ ID NO: 17 - DNA, 21 bp, synthetic construct
  misc_feature 1..21: note = Synthetic Construct
  source 1..21: mol_type = other DNA
acaatattcactgtgcccata

SEQ ID NO: 18 - DNA, 13 bp, synthetic construct
  misc_feature 1..13: note = Synthetic Construct
  misc_feature 3: note = locked nucleic acid
  misc_feature 5..6: note = locked nucleic acid
  misc_feature 8: note = locked nucleic acid
  misc_feature 10..11: note = locked nucleic acid
  source 1..13: mol_type = other DNA
tgacctacgaacc

SEQ ID NO: 19 - DNA, 17 bp, synthetic construct
  misc_feature 1..17: note = Synthetic Construct
  source 1..17: mol_type = other DNA
tgaggcgacactacgtc

SEQ ID NO: 20 - DNA, 23 bp, synthetic construct
  misc_feature 1..23: note = Synthetic Construct
  source 1..23: mol_type = other DNA
gtgcccattaataaatcttccaa

SEQ ID NO: 21 - DNA, 13 bp, synthetic construct
  misc_feature 1..13: note = Synthetic Construct
  misc_feature 3: note = locked nucleic acid
  misc_feature 5..6: note = locked nucleic acid
  misc_feature 9..10: note = locked nucleic acid
  source 1..13: mol_type = other DNA
agagcacacacat

SEQ ID NO: 22 - DNA, 13 bp, synthetic construct
  misc_feature 1..13: note = Synthetic Construct
  misc_feature 3: note = locked nucleic acid
  misc_feature 5..7: note = locked nucleic acid
  misc_feature 9..10: note = locked nucleic acid
  source 1..13: mol_type = other DNA
cacacgtagacat

SEQ ID NO: 23 - DNA, 17 bp, synthetic construct
  misc_feature 1..17: note = Synthetic Construct
  misc_feature 15: note = locked nucleic acid
  source 1..17: mol_type = other DNA
tgcaccaaaagagaact

SEQ ID NO: 24 - DNA, 19 bp, synthetic construct
  misc_feature 1..19: note = Synthetic Construct
  misc_feature 16: note = locked nucleic acid
  source 1..19: mol_type = other DNA
gtgcataactgtggtaact

SEQ ID NO: 25 - DNA, 13 bp, synthetic construct
  misc_feature 1..13: note = Synthetic Construct
  misc_feature 3..4: note = locked nucleic acid
  misc_feature 6: note = locked nucleic acid
  misc_feature 10: note = locked nucleic acid
  misc_feature 12: note = locked nucleic acid
  source 1..13: mol_type = other DNA
ctgtgggtcctga

SEQ ID NO: 26 - DNA, 21 bp, synthetic construct
  misc_feature 1..21: note = Synthetic Construct
  source 1..21: mol_type = other DNA
agagctgcaaacaactataca

SEQ ID NO: 27 - DNA, 18 bp, synthetic construct
  misc_feature 1..18: note = Synthetic Construct
  source 1..18: mol_type = other DNA
tatacctcacgtcgcagt

SEQ ID NO: 28 - DNA, 27 bp, synthetic construct
  misc_feature 1..27: note = Synthetic Construct
  source 1..27: mol_type = other DNA
agaatgtgtgtactgcaagcaacagtt

SEQ ID NO: 29 - DNA, 22 bp, synthetic construct
  misc_feature 1..22: note = Synthetic Construct
  source 1..22: mol_type = other DNA
cgtgaggtatatgactttgctt

SEQ ID NO: 30 - DNA, 22 bp, synthetic construct
  misc_feature 1..22: note = Synthetic Construct
  source 1..22: mol_type = other DNA
tcacatacagcatatggattcc

SEQ ID NO: 31 - DNA, 13 bp, synthetic construct
  misc_feature 1..13: note = Synthetic Construct
  misc_feature 3..4: note = locked nucleic acid
  misc_feature 7: note = locked nucleic acid
  misc_feature 10..12: note = locked nucleic acid
  source 1..13: mol_type = other DNA
cgggatttatgca

SEQ ID NO: 32 - DNA, 24 bp, synthetic construct
  misc_feature 1..24: note = Synthetic Construct
  misc_feature 22..23: note = locked nucleic acid
  source 1..24: mol_type = other DNA
gttttattctaaaattagtgagta

SEQ ID NO: 33 - DNA, 21 bp, synthetic construct
  misc_feature 1..21: note = Synthetic Construct
  misc_feature 16: note = locked nucleic acid
  source 1..21: mol_type = other DNA
ttgtattgctgttctaatgtt

SEQ ID NO: 34 - DNA, 12 bp, synthetic construct
  misc_feature 1..12: note = Synthetic Construct
  misc_feature 5..7: note = locked nucleic acid
  misc_feature 9..11: note = locked nucleic acid
  source 1..12: mol_type = other DNA
agtttgtatgga

SEQ ID NO: 35 - DNA, 20 bp, synthetic construct
  misc_feature 1..20: note = Synthetic Construct
  source 1..20: mol_type = other DNA
caaaccgttgtgtgatttgt

SEQ ID NO: 36 - DNA, 22 bp, synthetic construct
  misc_feature 1..22: note = Synthetic Construct
  source 1..22: mol_type = other DNA
gatgtctttgcttttcttcagg

SEQ ID NO: 37 - DNA, 12 bp, synthetic construct
  misc_feature 1..12: note = Synthetic Construct
  misc_feature 5..7: note = locked nucleic acid
  misc_feature 10..11: note = locked nucleic acid
  source 1..12: mol_type = other DNA
aagccactgtgt

SEQ ID NO: 38 - DNA, 18 bp, synthetic construct
  misc_feature 1..18: note = Synthetic Construct
  misc_feature 17: note = locked nucleic acid
  source 1..18: mol_type = other DNA
tctggacaaaaagcaaag

SEQ ID NO: 39 - DNA, 18 bp, synthetic construct
  misc_feature 1..18: note = Synthetic Construct
  misc_feature 3: note = locked nucleic acid
  source 1..18: mol_type = other DNA
gatgatctgcaacaagac

SEQ ID NO: 40 - DNA, 13 bp, synthetic construct
  misc_feature 1..13: note = Synthetic Construct
  misc_feature 6: note = locked nucleic acid
  misc_feature 8..9: note = locked nucleic acid
  source 1..13: mol_type = other DNA
tccaccgacccct

SEQ ID NO: 41 - DNA, 25 bp, synthetic construct
  misc_feature 1..25: note = Synthetic Construct
  source 1..25: mol_type = other DNA
tgcatgaatatatgttagatttgca

SEQ ID NO: 42 - DNA, 22 bp, synthetic construct
  misc_feature 1..22: note = Synthetic Construct
  source 1..22: mol_type = other DNA
tcctctgagctgtcatttaatt

SEQ ID NO: 43 - DNA, 13 bp, synthetic construct
  misc_feature 1..13: note = Synthetic Construct
  misc_feature 2..3: note = locked nucleic acid
  misc_feature 5..7: note = locked nucleic acid
  misc_feature 12: note = locked nucleic acid
  source 1..13: mol_type = other DNA
acaactgatctct

SEQ ID NO: 44 - DNA, 18 bp, synthetic construct
  misc_feature 1..18: note = Synthetic Construct
  misc_feature 4: note = locked nucleic acid
  source 1..18: mol_type = other DNA
tgaaatagatggtccagc

SEQ ID NO: 45 - DNA, 20 bp, synthetic construct
  misc_feature 1..20: note = Synthetic Construct
  misc_feature 18: note = locked nucleic acid
  source 1..20: mol_type = other DNA
tgcaacaaaaggttacaata

SEQ ID NO: 46 - DNA, 13 bp, synthetic construct
  misc_feature 1..13: note = Synthetic Construct
  misc_feature 4..5: note = locked nucleic acid
  misc_feature 8..9: note = locked nucleic acid
  misc_feature 11..12: note = locked nucleic acid
  source 1..13: mol_type = other DNA
cagagcccattac

SEQ ID NO: 47 - DNA, 19 bp, synthetic construct
  misc_feature 1..19: note = Synthetic Construct
  source 1..19: mol_type = other DNA
tgactctacgcttcggttg

SEQ ID NO: 48 - DNA, 19 bp, synthetic construct
  misc_feature 1..19: note = Synthetic Construct
  source 1..19: mol_type = other DNA
gcccattaacaggtcttcc

SEQ ID NO: 49 - DNA, 30 bp, synthetic construct
  misc_feature 1..30: note = Synthetic Construct
  source 1..30: mol_type = other DNA
tacaaagcacacacgtagacattcgtactt

SEQ ID NO: 50 - DNA, 30 bp, synthetic construct; identical to SEQ ID NO: 3
  misc_feature 1..30: note = Synthetic Construct
  source 1..30: mol_type = other DNA

SEQ ID NO: 51 - DNA, 13 bp, synthetic construct
  misc_feature 1..13: note = Synthetic Construct
  misc_feature 3: note = locked nucleic acid
  misc_feature 5..7: note = locked nucleic acid
  misc_feature 9..10: note = locked nucleic acid
  source 1..13: mol_type = other DNA
cacacgtagacat

SEQ ID NO: 52 - DNA, 17 bp, synthetic construct
  misc_feature 1..17: note = Synthetic Construct
  misc_feature 11: note = locked nucleic acid
  misc_feature 17: note = locked nucleic acid
  source 1..17: mol_type = other DNA
actgcaatgtttcagga

SEQ ID NO: 53 - DNA, 17 bp, synthetic construct
  misc_feature 1..17: note = Synthetic Construct
  misc_feature 4: note = locked nucleic acid
  misc_feature 7: note = locked nucleic acid
  misc_feature 10: note = locked nucleic acid
  misc_feature 16: note = locked nucleic acid
  source 1..17: mol_type = other DNA
catgtatagttgtttgc

SEQ ID NO: 54 - DNA, 28 bp, synthetic construct
  misc_feature 1..28: note = Synthetic Construct
  source 1..28: mol_type = other DNA
cgacccagaaagttaccacagttatgca

SEQ ID NO: 55 - DNA, 20 bp, synthetic construct
  misc_feature 1..20: note = Synthetic Construct
  misc_feature 19: note = locked nucleic acid
  source 1..20: mol_type = other DNA
ttagaatgtgtgtactgcaa

SEQ ID NO: 56 - DNA, 18 bp, synthetic construct
  misc_feature 1..18: note = Synthetic Construct
  misc_feature 10: note = locked nucleic acid
  source 1..18: mol_type = other DNA
cataaatcccgaaaagca

SEQ ID NO: 57 - DNA, 26 bp, synthetic construct
  misc_feature 1..26: note = Synthetic Construct
  source 1..26: mol_type = other DNA
gcaacagttactgcgacgtgaggtat

SEQ ID NO: 58 - DNA, 20 bp, synthetic construct
  misc_feature 1..20: note = Synthetic Construct
  misc_feature 5: note = locked nucleic acid
  misc_feature 11: note = locked nucleic acid
  misc_feature 15: note = locked nucleic acid
  source 1..20: mol_type = other DNA
catagtatatagagatggga

SEQ ID NO: 59 - DNA, 20 bp, synthetic construct
  misc_feature 1..20: note = Synthetic Construct
  misc_feature 3: note = locked nucleic acid
  misc_feature 8: note = locked nucleic acid
  misc_feature 11: note = locked nucleic acid
  misc_feature 18: note = locked nucleic acid
  source 1..20: mol_type = other DNA
tctatactcactaattttag

SEQ ID NO: 60 - DNA, 12 bp, synthetic construct
  misc_feature 1..12: note = Synthetic Construct
  misc_feature 2..3: note = locked nucleic acid
  misc_feature 5..6: note = locked nucleic acid
  misc_feature 9..10: note = locked nucleic acid
  source 1..12: mol_type = other DNA
atcacatacagc

SEQ ID NO: 61 - DNA, 20 bp, synthetic construct
  misc_feature 1..20: note = Synthetic Construct
  misc_feature 14..15: note = locked nucleic acid
  misc_feature 17..18: note = locked nucleic acid
  source 1..20: mol_type = other DNA
cattattgttatagtttgta

SEQ ID NO: 62 - DNA, 21 bp, synthetic construct
  misc_feature 1..21: note = Synthetic Construct
  misc_feature 17: note = locked nucleic acid
  source 1..21: mol_type = other DNA
taattaacaaatcacacaacg

SEQ ID NO: 63 - DNA, 13 bp, synthetic construct
  misc_feature 1..13: note = Synthetic Construct
  misc_feature 3..6: note = locked nucleic acid
  misc_feature 8: note = locked nucleic acid
  misc_feature 11: note = locked nucleic acid
  source 1..13: mol_type = other DNA
tatggaacaacat

SEQ ID NO: 64 - DNA, 18 bp, synthetic construct
  misc_feature 1..18: note = Synthetic Construct
  misc_feature 3: note = locked nucleic acid
  misc_feature 9: note = locked nucleic acid
  misc_feature 11: note = locked nucleic acid
  misc_feature 14: note = locked nucleic acid
  source 1..18: mol_type = other DNA
tgtattaactgtcaaaag

SEQ ID NO: 65 - DNA, 18 bp, synthetic construct
  misc_feature 1..18: note = Synthetic Construct
  misc_feature 4: note = locked nucleic acid
  misc_feature 16: note = locked nucleic acid
  source 1..18: mol_type = other DNA
ggaatctttgctttttgt

SEQ ID NO: 66 - DNA, 13 bp, synthetic construct
  misc_feature 1..13: note = Synthetic Construct
  misc_feature 3..4: note = locked nucleic acid
  misc_feature 9..10: note = locked nucleic acid
  misc_feature 12: note = locked nucleic acid
  source 1..13: mol_type = other DNA
tgtgtcctgaaga

SEQ ID NO: 67 - DNA, 19 bp, synthetic construct
  misc_feature 1..19: note = Synthetic Construct
  misc_feature 17: note = locked nucleic acid
  source 1..19: mol_type = other DNA
ataatataaggggtcggtg

SEQ ID NO: 68 - DNA, 17 bp, synthetic construct
  misc_feature 1..17: note = Synthetic Construct
  source 1..17: mol_type = other DNA
agctgggtttctctacg

SEQ ID NO: 69 - DNA, 30 bp, synthetic construct
  misc_feature 1..30: note = Synthetic Construct
  source 1..30: mol_type = other DNA
cggtcgatgtatgtcttgttgcagatcatc

SEQ ID NO: 70 - DNA, 27 bp, synthetic construct
  misc_feature 1..27: note = Synthetic Construct
  source 1..27: mol_type = other DNA
ccggtcgatgtatgtcttgttgcagat

SEQ ID NO: 71 - DNA, 17 bp, synthetic construct
  misc_feature 1..17: note = Synthetic Construct
  source 1..17: mol_type = other DNA
tgcatggagatacacct

SEQ ID NO: 72 - DNA, 18 bp, synthetic construct
  misc_feature 1..18: note = Synthetic Construct
  source 1..18: mol_type = other DNA
acagtagagatcagttgt

SEQ ID NO: 73 - DNA, 12 bp, synthetic construct
  misc_feature 1..12: note = Synthetic Construct
  misc_feature 3: note = locked nucleic acid
  misc_feature 5..6: note = locked nucleic acid
  misc_feature 8..9: note = locked nucleic acid
  misc_feature 11: note = locked nucleic acid
  source 1..12: mol_type = other DNA
ccagagacaact

SEQ ID NO: 74 - DNA, 19 bp, synthetic construct
  misc_feature 1..19: note = Synthetic Construct
  misc_feature 14..15: note = locked nucleic acid
  misc_feature 17: note = locked nucleic acid
  source 1..19: mol_type = other DNA
tatgagcaattaaatgaca

SEQ ID NO: 75 - DNA, 18 bp, synthetic construct
  misc_feature 1..18: note = Synthetic Construct
  misc_feature 6: note = locked nucleic acid
  source 1..18: mol_type = other DNA
attgtaatgggctctgtc

SEQ ID NO: 76 - DNA, 13 bp, synthetic construct
  misc_feature 1..13: note = Synthetic Construct
  misc_feature 5..6: note = locked nucleic acid
  misc_feature 9..12: note = locked nucleic acid
  source 1..13: mol_type = other DNA
atttcatcctcct

SEQ ID NO: 77 - DNA, 18 bp, synthetic construct
  misc_feature 1..18: note = Synthetic Construct
  misc_feature 4: note = locked nucleic acid
  source 1..18: mol_type = other DNA
tacaaagcacacacgtag

SEQ ID NO: 78 - DNA, 21 bp, synthetic construct
  misc_feature 1..21: note = Synthetic Construct
  misc_feature 3: note = locked nucleic acid
  source 1..21: mol_type = other DNA
ttatggtttctgagaacagat

SEQ ID NO: 79 - DNA, 25 bp, synthetic construct
  misc_feature 1..25: note = Synthetic Construct
  source 1..25: mol_type = other DNA
tggaagacctgttaatgggcacact

SEQ ID NO: 80 - DNA, 17 bp, synthetic construct
  misc_feature 1..17: note = Synthetic Construct
  source 1..17: mol_type = other DNA
cgctttgaggatccaac

SEQ ID NO: 81 - DNA, 18 bp, synthetic construct
  misc_feature 1..18: note = Synthetic Construct
  source 1..18: mol_type = other DNA
gcagtgaagtgttcagtt

SEQ ID NO: 82 - DNA, 25 bp, synthetic construct
  misc_feature 1..25: note = Synthetic Construct
  source 1..25: mol_type = other DNA
accctacaagctacctgatctgtgc

SEQ ID NO: 83 - DNA, 20 bp, synthetic construct
  misc_feature 1..20: note = Synthetic Construct
  misc_feature 7: note = locked nucleic acid
  misc_feature 19: note = locked nucleic acid
  source 1..20: mol_type = other DNA
aagacatagaaataacctgt

SEQ ID NO: 84 - DNA, 18 bp, synthetic construct
  misc_feature 1..18: note = Synthetic Construct
  misc_feature 5..8: note = locked nucleic acid
  source 1..18: mol_type = other DNA
ttaaatgcaaattcaaat

SEQ ID NO: 85 - DNA, 29 bp, synthetic construct
  misc_feature 1..29: note = Synthetic Construct
  source 1..29: mol_type = other DNA
tgcaagacagtattggaacttacagaggt

SEQ ID NO: 86 - DNA, 20 bp, synthetic construct
  misc_feature 1..20: note = Synthetic Construct
  misc_feature 5: note = locked nucleic acid
  source 1..20: mol_type = other DNA
ttatttgtggtgtatagaga

SEQ ID NO: 87 - DNA, 21 bp, synthetic construct
  misc_feature 1..21: note = Synthetic Construct
  misc_feature 5: note = locked nucleic acid
  misc_feature 7: note = locked nucleic acid
  misc_feature 13: note = locked nucleic acid
  source 1..21: mol_type = other DNA
aattctctaattctagaataa

SEQ ID NO: 88 - DNA, 13 bp, synthetic construct
  misc_feature 1..13: note = Synthetic Construct
  misc_feature 3: note = locked nucleic acid
  misc_feature 5..8: note = locked nucleic acid
  misc_feature 10: note = locked nucleic acid
  source 1..13: mol_type = other DNA
catgcggtatact

SEQ ID NO: 89 - DNA, 19 bp, synthetic construct
  misc_feature 1..19: note = Synthetic Construct
  misc_feature 6: note = locked nucleic acid
  misc_feature 10: note = locked nucleic acid
  misc_feature 17: note = locked nucleic acid
  source 1..19: mol_type = other DNA
aagacattattcagactct

SEQ ID NO: 90 - DNA, 18 bp, synthetic construct
  misc_feature 1..18: note = Synthetic Construct
  misc_feature 10: note = locked nucleic acid
  misc_feature 16..17: note = locked nucleic acid
  source 1..18: mol_type = other DNA
aataaattgtataaccca

SEQ ID NO: 91 - DNA, 12 bp, synthetic construct
  misc_feature 1..12: note = Synthetic Construct
  misc_feature 3..4: note = locked nucleic acid
  misc_feature 7..10: note = locked nucleic acid
  source 1..12: mol_type = other DNA
tggagacacatt

SEQ ID NO: 92 - DNA, 18 bp, synthetic construct
  misc_feature 1..18: note = Synthetic Construct
  source 1..18: mol_type = other DNA
agaaaccgttgaatccag

SEQ ID NO: 93 - DNA, 19 bp, synthetic construct
  misc_feature 1..19: note = Synthetic Construct
  source 1..19: mol_type = other DNA
atttcacaacatagctggg

SEQ ID NO: 94 - DNA, 14 bp, synthetic construct
  misc_feature 1..14: note = Synthetic Construct
  misc_feature 3: note = locked nucleic acid
  misc_feature 6..8: note = locked nucleic acid
  misc_feature 11..12: note = locked nucleic acid
  source 1..14: mol_type = other DNA
agacaccttaatga

SEQ ID NO: 95 - DNA, 16 bp, synthetic construct
  misc_feature 1..16: note = Synthetic Construct
  source 1..16: mol_type = other DNA
ccagtgccattcgtgc

SEQ ID NO: 96 - DNA, 19 bp, synthetic construct
  misc_feature 1..19: note = Synthetic Construct
  misc_feature 6: note = locked nucleic acid
  misc_feature 10: note = locked nucleic acid
  source 1..19: mol_type = other DNA
ttatacttgtgtttctctg

SEQ ID NO: 97 - DNA, 24 bp, synthetic construct
  misc_feature 1..24: note = Synthetic Construct
  source 1..24: mol_type = other DNA
cacgacaggaacgactccaacgac

SEQ ID NO: 98 - DNA, 17 bp, synthetic construct
  misc_feature 1..17: note = Synthetic Construct
  source 1..17: mol_type = other DNA
atggacctaaggcaaca

SEQ ID NO: 99 - DNA, 18 bp, synthetic construct
  misc_feature 1..18: note = Synthetic Construct
  misc_feature 3: note = locked nucleic acid
  source 1..18: mol_type = other DNA
tgacatagaaggtcaacc

SEQ ID NO: 100 - DNA, 11 bp, synthetic construct
  misc_feature 1..11: note = Synthetic Construct
  misc_feature 3: note = locked nucleic acid
  misc_feature 5..8: note = locked nucleic acid
  misc_feature 10: note = locked nucleic acid
  source 1..11: mol_type = other DNA
tttagagcccc

SEQ ID NO: 101 - DNA, 18 bp, synthetic construct
  misc_feature 1..18: note = Synthetic Construct
  misc_feature 8: note = locked nucleic acid
  source 1..18: mol_type = other DNA
cgagcaattaagcgactc

SEQ ID NO: 102 - DNA, 18 bp, synthetic construct
  misc_feature 1..18: note = Synthetic Construct
  source 1..18: mol_type = other DNA
cgggctggtaaatgttga

SEQ ID NO: 103 - DNA, 13 bp, synthetic construct
  misc_feature 1..13: note = Synthetic Construct
  misc_feature 2..4: note = locked nucleic acid
  misc_feature 8: note = locked nucleic acid
  misc_feature 11..12: note = locked nucleic acid
  source 1..13: mol_type = other DNA
tcgttttcttcct

SEQ ID NO: 104 - DNA, 18 bp, synthetic construct
  misc_feature 1..18: note = Synthetic Construct
  source 1..18: mol_type = other DNA
acaacgtcacacaatgtt

SEQ ID NO: 105 - DNA, 18 bp, synthetic construct
  misc_feature 1..18: note = Synthetic Construct
  source 1..18: mol_type = other DNA
tctgctgagctttctact

SEQ ID NO: 106 - DNA, 29 bp, synthetic construct
  misc_feature 1..29: note = Synthetic Construct
  source 1..29: mol_type = other DNA
tgtatgtgttgtaagtgtgaagccagaat

SEQ ID NO: 107 - DNA, 16 bp, synthetic construct
  misc_feature 1..16: note = Synthetic Construct
  source 1..16: mol_type = other DNA
accttcgagcattcca

SEQ ID NO: 108 - DNA, 16 bp, synthetic construct
  misc_feature 1..16: note = Synthetic Construct
  source 1..16: mol_type = other DNA
ttactgctgggatgca

SEQ ID NO: 109 - DNA, 13 bp, synthetic construct
  misc_feature 1..13: note = Synthetic Construct
  misc_feature 6..7: note = locked nucleic acid
  misc_feature 9: note = locked nucleic acid
  misc_feature 11..12: note = locked nucleic acid
  source 1..13: mol_type = other DNA
ctgaacaccctgt

SEQ ID NO: 110 - DNA, 18 bp, synthetic construct
  misc_feature 1..18: note = Synthetic Construct
  source 1..18: mol_type = other DNA
ccctacaagctacctgat

SEQ ID NO: 111 - DNA, 19 bp, synthetic construct
  misc_feature 1..19: note = Synthetic Construct
  misc_feature 8: note = locked nucleic acid
  misc_feature 10: note = locked nucleic acid
  misc_feature 13: note = locked nucleic acid
  misc_feature 15: note = locked nucleic acid
  source 1..19: mol_type = other DNA
caatatacacaggttattt

SEQ ID NO: 112 - DNA, 13 bp, synthetic construct
  misc_feature 1..13: note = Synthetic Construct
  misc_feature 3..5: note = locked nucleic acid
  misc_feature 8..9: note = locked nucleic acid
  source 1..13: mol_type = other DNA
cacggaactgaac

SEQ ID NO: 113 - DNA, 18 bp, synthetic construct
  misc_feature 1..18: note = Synthetic Construct
  misc_feature 6..7: note = locked nucleic acid
  misc_feature 12..13: note = locked nucleic acid
  misc_feature 16: note = locked nucleic acid
  source 1..18: mol_type = other DNA
tatttgaatttgcattta

SEQ ID NO: 114 - DNA, 18 bp, synthetic construct
  misc_feature 1..18: note = Synthetic Construct
  misc_feature 4: note = locked nucleic acid
  misc_feature 9..10: note = locked nucleic acid
  misc_feature 16: note = locked nucleic acid
  source 1..18: mol_type = other DNA
aatctatacatttatggc

SEQ ID NO: 115 - DNA, 14 bp, synthetic construct
  misc_feature 1..14: note = Synthetic Construct
  misc_feature 3: note = locked nucleic acid
  misc_feature 5: note = locked nucleic acid
  misc_feature 7: note = locked nucleic acid
  misc_feature 9: note = locked nucleic acid
  misc_feature 12: note = locked nucleic acid
  source 1..14: mol_type = other DNA
agacagtataccgc

SEQ ID NO: 116 - DNA, 20 bp, synthetic construct
  misc_feature 1..20: note = Synthetic Construct
  misc_feature 4: note = locked nucleic acid
  misc_feature 10..12: note = locked nucleic acid
  misc_feature 17: note = locked nucleic acid
  source 1..20: mol_type = other DNA
ctagaattagagaattaaga

SEQ ID NO: 117 - DNA, 22 bp, synthetic construct
  misc_feature 1..22: note = Synthetic Construct
  misc_feature 16: note = locked nucleic acid
  source 1..22: mol_type = other DNA
agtgttagttagtttttccaat

SEQ ID NO: 118 - DNA, 13 bp, synthetic construct
  misc_feature 1..13: note = Synthetic Construct
  misc_feature 3..6: note = locked nucleic acid
  misc_feature 8: note = locked nucleic acid
  misc_feature 11: note = locked nucleic acid
  source 1..13: mol_type = other DNA
tcagactctgtgt

SEQ ID NO: 119 - DNA, 17 bp, synthetic construct
  misc_feature 1..17: note = Synthetic Construct
  misc_feature 5: note = locked nucleic acid
  misc_feature 15: note = locked nucleic acid
  source 1..17: mol_type = other DNA
attaataaggtgcctgc

SEQ ID NO: 120 - DNA, 19 bp, synthetic construct
  misc_feature 1..19: note = Synthetic Construct
  misc_feature 14: note = locked nucleic acid
  source 1..19: mol_type = other DNA
tcgtttttcattaaggtgt

SEQ ID NO: 121 - DNA, 13 bp, synthetic construct
  misc_feature 1..13: note = Synthetic Construct
  misc_feature 6..8: note = locked nucleic acid
  misc_feature 11..12: note = locked nucleic acid
  source 1..13: mol_type = other DNA
tgaatccagcaga

SEQ ID NO: 122 - DNA, 19 bp, synthetic construct
  misc_feature 1..19: note = Synthetic Construct
  source 1..19: mol_type = other DNA
atttcacaacatagctggg

SEQ ID NO: 123 - DNA, 17 bp, synthetic construct
  misc_feature 1..17: note = Synthetic Construct
  source 1..17: mol_type = other DNA
gtttctctgcgtcgttg

SEQ ID NO: 124 - DNA, 13 bp, synthetic construct
  misc_feature 1..13: note = Synthetic Construct
  misc_feature 3: note = locked nucleic acid
  misc_feature 5..8: note = locked nucleic acid
  misc_feature 11: note = locked nucleic acid
  source 1..13: mol_type = other DNA
agtgccattcgtg

SEQ ID NO: 125 - DNA, 20 bp, synthetic construct
  misc_feature 1..20: note = Synthetic Construct
  misc_feature 4: note = locked nucleic acid
  source 1..20: mol_type = other DNA
attgtattgcatttagagcc

SEQ ID NO: 126 - DNA, 18 bp, synthetic construct
  misc_feature 1..18: note = Synthetic Construct
  misc_feature 16: note = locked nucleic acid
  source 1..18: mol_type = other DNA
ttcatcgttttcttcctc

SEQ ID NO: 127 - DNA, 13 bp, synthetic construct
  misc_feature 1..13: note = Synthetic Construct
  misc_feature 7..9: note = locked nucleic acid
  misc_feature 9..11: note = locked nucleic acid
  source 1..13: mol_type = other DNA
ctatgtcacgagc

SEQ ID NO: 128 - DNA, 20 bp, synthetic construct
  misc_feature 1..20: note = Synthetic Construct
  misc_feature 8: note = locked nucleic acid
  misc_feature 14: note = locked nucleic acid
  source 1..20: mol_type = other DNA
atagatggagttaatcatca

SEQ ID NO: 129 - DNA, 18 bp, synthetic construct
  misc_feature 1..18: note = Synthetic Construct
  misc_feature 3: note = locked nucleic acid
  misc_feature 13: note = locked nucleic acid
  source 1..18: mol_type = other DNA
acttacaacacatacaca

SEQ ID NO: 130 - DNA, 25 bp, synthetic construct
  misc_feature 1..25: note = Synthetic Construct
  source 1..25: mol_type = other DNA
ccgaaccacaacgtcacacaatgtt

SEQ ID NO: 131 - DNA, 20 bp, synthetic construct
  misc_feature 1..20: note = Synthetic Construct
  source 1..20: mol_type = other DNA
tgaagccagaattgagctag

SEQ ID NO: 132 - DNA, 18 bp, synthetic construct
  misc_feature 1..18: note = Synthetic Construct
  source 1..18: mol_type = other DNA
aggacagggtgttcagaa

SEQ ID NO: 133 - DNA, 13 bp, synthetic construct
  misc_feature 1..13: note = Synthetic Construct
  misc_feature 3: note = locked nucleic acid
  misc_feature 5..6: note = locked nucleic acid
  misc_feature 9: note = locked nucleic acid
  source 1..13: mol_type = other DNA
cagacgaccttcg

SEQ ID NO: 134 - DNA, 18 bp, synthetic construct
  misc_feature 1..18: note = Synthetic Construct
  misc_feature 12: note = locked nucleic acid
  source 1..18: mol_type = other DNA
atgttcaaaaatcctgca

SEQ ID NO: 135 - DNA, 19 bp, synthetic construct
  misc_feature 1..19: note = Synthetic Construct
  misc_feature 16: note = locked nucleic acid
  source 1..19: mol_type = other DNA
ttcatcgtagggtatttcc

SEQ ID NO: 136 - DNA, 13 bp, synthetic construct
  misc_feature 1..13: note = Synthetic Construct
  misc_feature 4..5: note = locked nucleic acid
  misc_feature 8..9: note = locked nucleic acid
  misc_feature 11..12: note = locked nucleic acid
  source 1..13: mol_type = other DNA
aactaagctcggc

SEQ ID NO: 137 - DNA, 19 bp, synthetic construct
  misc_feature 1..19: note = Synthetic Construct
  misc_feature 3: note = locked nucleic acid
  misc_feature 11: note = locked nucleic acid
  misc_feature 18: note = locked nucleic acid
  source 1..19: mol_type = other DNA
ctaagattgaattgtgtct

SEQ ID NO: 138 - DNA, 23 bp, synthetic construct
  misc_feature 1..23: note = Synthetic Construct
  misc_feature 7: note = locked nucleic acid
  misc_feature 18: note = locked nucleic acid
  source 1..23: mol_type = other DNA
taaatctgtaaatgcaaaatcta

SEQ ID NO: 139 - DNA, 14 bp, synthetic construct
  misc_feature 1..14: note = Synthetic Construct
  misc_feature 3: note = locked nucleic acid
  misc_feature 6: note = locked nucleic acid
  misc_feature 8: note = locked nucleic acid
  misc_feature 10..11: note = locked nucleic acid
  misc_feature 13: note = locked nucleic acid
  source 1..14: mol_type = other DNA
acagaaacagaggt

SEQ ID NO: 140 - DNA, 21 bp, synthetic construct
  misc_feature 1..21: note = Synthetic Construct
  misc_feature 7: note = locked nucleic acid
  source 1..21: mol_type = other DNA
acaatagtatatagggacgac

SEQ ID NO: 141 - DNA, 22 bp, synthetic construct
  misc_feature 1..22: note = Synthetic Construct
  misc_feature 7: note = locked nucleic acid
  misc_feature 16: note = locked nucleic acid
  misc_feature 19: note = locked nucleic acid
  source 1..22: mol_type = other DNA
ttcacttacttttgaataaaat

SEQ ID NO: 142 - DNA, 13 bp, synthetic construct
  misc_feature 1..13: note = Synthetic Construct
  misc_feature 3..5: note = locked nucleic acid
  misc_feature 9..10: note = locked nucleic acid
  source 1..13: mol_type = other DNA
acggagtgtgtac

SEQ ID NO: 143 - DNA, 23 bp, synthetic construct
  misc_feature 1..23: note = Synthetic Construct
  misc_feature 5: note = locked nucleic acid
  misc_feature 9: note = locked nucleic acid
  source 1..23: mol_type = other DNA
tttagatggtatagatatagtgt

SEQ ID NO: 144 - DNA, 20 bp, synthetic construct
  misc_feature 1..20: note = Synthetic Construct
  misc_feature 3: note = locked nucleic acid
  misc_feature 10..11: note = locked nucleic acid
  source 1..20: mol_type = other DNA
cctaattaacaaatcacata

SEQ ID NO: 145 - DNA, 13 bp, synthetic construct
  misc_feature 1..13: note = Synthetic Construct
  misc_feature 2..5: note = locked nucleic acid
  misc_feature 7..8: note = locked nucleic acid
  source 1..13: mol_type = other DNA
atggaacaacatt

SEQ ID NO: 146 - DNA, 19 bp, synthetic construct
  misc_feature 1..19: note = Synthetic Construct
  misc_feature 6: note = locked nucleic acid
  misc_feature 13: note = locked nucleic acid
  source 1..19: mol_type = other DNA
tgtataacgtgtcaaagac

SEQ ID NO: 147 - DNA, 18 bp, synthetic construct
  misc_feature 1..18: note = Synthetic Construct
  misc_feature 11: note = locked nucleic acid
  misc_feature 14: note = locked nucleic acid
  source 1..18: mol_type = other DNA
ttgtggaatcgtttcttt

SEQ ID NO: 148 - DNA, 13 bp, synthetic construct
  misc_feature 1..13: note = Synthetic Construct
  misc_feature 4..5: note = locked nucleic acid
  misc_feature 7..8: note = locked nucleic acid
  misc_feature 11..12: note = locked nucleic acid
  source 1..13: mol_type = other DNA
tgtgtccagaaga

SEQ ID NO: 149 - DNA, 18 bp, synthetic construct
  misc_feature 1..18: note = Synthetic Construct
  source 1..18: mol_type = other DNA
cataggaggaaggtggac

SEQ ID NO: 150 - DNA, 17 bp, synthetic construct
  misc_feature 1..17: note = Synthetic Construct
  misc_feature 9: note = locked nucleic acid
  misc_feature 13: note = locked nucleic acid
  source 1..17: mol_type = other DNA
ttacacttgggtttcag

SEQ ID NO: 151 - DNA, 26 bp, synthetic construct
  misc_feature 1..26: note = Synthetic Construct
  source 1..26: mol_type = other DNA
cgttgcatagcatgttggagaagacc

SEQ ID NO: 152 - DNA, 19 bp, synthetic construct
  misc_feature 1..19: note = Synthetic Construct
  misc_feature 6: note = locked nucleic acid
  misc_feature 16: note = locked nucleic acid
  source 1..19: mol_type = other DNA
caagactatgtgttagatt

SEQ ID NO: 153 - DNA, 22 bp, synthetic construct
  misc_feature 1..22: note = Synthetic Construct
  misc_feature 14: note = locked nucleic acid
  misc_feature 17: note = locked nucleic acid
  source 1..22: mol_type = other DNA
tcatctgagctgtcgggtaatt

SEQ ID NO: 154 - DNA, 13 bp, synthetic construct
  misc_feature 1..13: note = Synthetic Construct
  misc_feature 7..9: note = locked nucleic acid
  misc_feature 11..12: note = locked nucleic acid
  source 1..13: mol_type = other DNA
aactgacctccac

SEQ ID NO: 155 - DNA, 18 bp, synthetic construct
  misc_feature 1..18: note = Synthetic Construct
  misc_feature 12: note = locked nucleic acid
  source 1..18: mol_type = other DNA
aggatgtcatagacagtc

SEQ ID NO: 156 - DNA, 19 bp, synthetic construct
  misc_feature 1..19: note = Synthetic Construct
  misc_feature 3: note = locked nucleic acid
  source 1..19: mol_type = other DNA
tgtagacttacactgacaa

SEQ ID NO: 157 - DNA, 13 bp, synthetic construct
  misc_feature 1..13: note = Synthetic Construct
  misc_feature 4..5: note = locked nucleic acid
  misc_feature 8: note = locked nucleic acid
  misc_feature 10..11: note = locked nucleic acid
  source 1..13: mol_type = other DNA
ctggacaagcaga

SEQ ID NO: 158 - DNA, 21 bp, synthetic construct
  misc_feature 1..21: note = Synthetic Construct
  source 1..21: mol_type = other DNA
agcacacaagtagatattcgc

SEQ ID NO: 159 - DNA, 19 bp, synthetic construct
  misc_feature 1..19: note = Synthetic Construct
  source 1..19: mol_type = other DNA
tagtagaacagttggggca

SEQ ID NO: 160 - DNA, 13 bp, synthetic construct
  misc_feature 1..13: note = Synthetic Construct
  misc_feature 4..5: note = locked nucleic acid
  misc_feature 7: note = locked nucleic acid
  misc_feature 9..10: note = locked nucleic acid
  source 1..13: mol_type = other DNA
taacagctcttgc

SEQ ID NO: 161 - DNA, 18 bp, synthetic construct
  misc_feature 1..18: note = Synthetic Construct
  misc_feature 10: note = locked nucleic acid
  misc_feature 16: note = locked nucleic acid
  source 1..18: mol_type = other DNA
aaattgcatgaactaagc

SEQ ID NO: 162 - DNA, 18 bp, synthetic construct
  misc_feature 1..18: note = Synthetic Construct
  misc_feature 3: note = locked nucleic acid
  source 1..18: mol_type = other DNA
ttaactgacctttgcagt

SEQ ID NO: 163 - DNA, 30 bp, synthetic construct
  misc_feature 1..30: note = Synthetic Construct
  source 1..30: mol_type = other DNA
cggcattggaaataccctacgatgaactaa

SEQ ID NO: 164 - DNA, 20 bp, synthetic construct
  misc_feature 1..20: note = Synthetic Construct
  misc_feature 6: note = locked nucleic acid
  misc_feature 18: note = locked nucleic acid
  source 1..20: mol_type = other DNA
cagaaacagaggtattagat

SEQ ID NO: 165 - DNA, 20 bp, synthetic construct
  misc_feature 1..20: note = Synthetic Construct
  misc_feature 4: note = locked nucleic acid
  misc_feature 17: note = locked nucleic acid
  source 1..20: mol_type = other DNA
ttaaacattttgtacacact

SEQ ID NO: 166 - DNA, 13 bp, synthetic construct
  misc_feature 1..13: note = Synthetic Construct
  misc_feature 3..5: note = locked nucleic acid
  misc_feature 7..8: note = locked nucleic acid
  source 1..13: mol_type = other DNA
acgacacaccaca

SEQ ID NO: 167 - DNA, 21 bp, synthetic construct
  misc_feature 1..21: note = Synthetic Construct
  misc_feature 5: note = locked nucleic acid
  misc_feature 12: note = locked nucleic acid
  misc_feature 17: note = locked nucleic acid
  source 1..21: mol_type = other DNA
attttattcaaaagtaagtga

SEQ ID NO: 168 - DNA, 20 bp, synthetic construct
  misc_feature 1..20: note = Synthetic Construct
  misc_feature 4: note = locked nucleic acid
  misc_feature 13: note = locked nucleic acid
  misc_feature 17: note = locked nucleic acid
  source 1..20: mol_type = other DNA
cctttgtttgtcaatttttc

SEQ ID NO: 169 - DNA, 13 bp, synthetic construct
  misc_feature 1..13: note = Synthetic Construct
  misc_feature 4..6: note = locked nucleic acid
  misc_feature 10..12: note = locked nucleic acid
  source 1..13: mol_type = other DNA
tagtgtgtatgga

SEQ ID NO: 170 - DNA, 23 bp, synthetic construct
  misc_feature 1..23: note = Synthetic Construct
  misc_feature 17: note = locked nucleic acid
  misc_feature 21: note = locked nucleic acid
  source 1..23: mol_type = other DNA
tatatgtgatttgttaattaggt

SEQ ID NO: 171 - DNA, 20 bp, synthetic construct
  misc_feature 1..20: note = Synthetic Construct
  misc_feature 6: note = locked nucleic acid
  misc_feature 11: note = locked nucleic acid
  source 1..20: mol_type = other DNA
tccaaatgtctttgtttttc

SEQ ID NO: 172 - DNA, 13 bp, synthetic construct
  misc_feature 1..13: note = Synthetic Construct
  misc_feature 3: note = locked nucleic acid
  misc_feature 6: note = locked nucleic acid
  misc_feature 8..11: note = locked nucleic acid
  source 1..13: mol_type = other DNA
ccgttgtgtccag

SEQ ID NO: 173 - DNA, 19 bp, synthetic construct
  misc_feature 1..19: note = Synthetic Construct
  misc_feature 6..16: note = locked nucleic acid
  misc_feature 7: note = locked nucleic acid
  source 1..19: mol_type = other DNA
taaaaagaaacgattccac

SEQ ID NO: 174 - DNA, 18 bp, synthetic construct
  misc_feature 1..18: note = Synthetic Construct
  misc_feature 3: note = locked nucleic acid
  source 1..18: mol_type = other DNA
tttcagtacgaggtcttc

SEQ ID NO: 175 - DNA, 20 bp, synthetic construct
  misc_feature 1..20: note = Synthetic Construct
  source 1..20: mol_type = other DNA
aaggtggacaggacgttgca

SEQ ID NO: 176 - DNA, 17 bp, synthetic construct
  misc_feature 1..17: note = Synthetic Construct
  source 1..17: mol_type = other DNA
tggagaaacacctacgt

SEQ ID NO: 177 - DNA, 20 bp, synthetic construct
  misc_feature 1..20: note = Synthetic Construct
  misc_feature 12: note = locked nucleic acid
  source 1..20: mol_type = other DNA
taattgctcataacagtgga

SEQ ID NO: 178 - DNA, 13 bp, synthetic construct
  misc_feature 1..13: note = Synthetic Construct
  misc_feature 3..6: note = locked nucleic acid
  source 1..13: mol_type = other DNA
aacctgaggcaac

SEQ ID NO: 179 - DNA, 18 bp, synthetic construct
  misc_feature 1..18: note = Synthetic Construct
  misc_feature 17: note = locked nucleic acid
  source 1..18: mol_type = other DNA
agatgaggaggatgtcat

SEQ ID NO: 180 - DNA, 19 bp, synthetic construct
  misc_feature 1..19: note = Synthetic Construct
  misc_feature 3: note = locked nucleic acid
  misc_feature 7: note = locked nucleic acid
  misc_feature 14: note = locked nucleic acid
  source 1..19: mol_type = other DNA
aggtaacgatattgtaatt

SEQ ID NO: 181 - DNA, 12 bp, synthetic construct
  misc_feature 1..12: note = Synthetic Construct
  misc_feature 3..6: note = locked nucleic acid
  misc_feature 8: note = locked nucleic acid
  misc_feature 11: note = locked nucleic acid
  source 1..12: mol_type = other DNA
caagcagaaccg

SEQ ID NO: 182 - DNA, 18 bp, synthetic construct
  misc_feature 1..18: note = Synthetic Construct
  misc_feature 8: note = locked nucleic acid
  misc_feature 15: note = locked nucleic acid
  source 1..18: mol_type = other DNA
tgtcagtgtaagtctaca

SEQ ID NO: 183 - DNA, 18 bp, synthetic construct
  misc_feature 1..18: note = Synthetic Construct
  misc_feature 14: note = locked nucleic acid
  source 1..18: mol_type = other DNA
tccaaatgagcccattaa

SEQ ID NO: 184 - DNA, 13 bp, synthetic construct
  misc_feature 1..13: note = Synthetic Construct
  misc_feature 4..7: note = locked nucleic acid
  misc_feature 9: note = locked nucleic acid
  misc_feature 12: note = locked nucleic acid
  source 1..13: mol_type = other DNA
tgtacagagcaca

SEQ ID NO: 185 - DNA, 18 bp, synthetic construct
  misc_feature 1..18: note = Synthetic Construct
  misc_feature 16: note = locked nucleic acid
  source 1..18: mol_type = other DNA
ttcaagacactgaggaaa

SEQ ID NO: 186 - DNA, 21 bp, synthetic construct
  misc_feature 1..21: note = Synthetic Construct
  misc_feature 9: note = locked nucleic acid
  misc_feature 17: note = locked nucleic acid
  source 1..21: mol_type = other DNA
aatgttgtgtatagttgtctc

SEQ ID NO: 187 - DNA, 27 bp, synthetic construct
  misc_feature 1..27: note = Synthetic Construct
  source 1..27: mol_type = other DNA
aacattgcatgatttgtgccaagcatt

SEQ ID NO: 188 - DNA, 18 bp, synthetic construct
  misc_feature 1..18: note = Synthetic Construct
  misc_feature 16: note = locked nucleic acid
  source 1..18: mol_type = other DNA
aatgcaaaaaacctttgc

SEQ ID NO: 189 - DNA, 19 bp, synthetic construct
  misc_feature 1..19: note = Synthetic Construct
  misc_feature 5: note = locked nucleic acid
  misc_feature 10: note = locked nucleic acid
  misc_feature 17: note = locked nucleic acid
  source 1..19: mol_type = other DNA
tccctctctatatacaact

SEQ ID NO: 190 - DNA, 13 bp, synthetic construct
  misc_feature 1..13: note = Synthetic Construct
  misc_feature 3: note = locked nucleic acid
  misc_feature 6..8: note = locked nucleic acid
  misc_feature 11..12: note = locked nucleic acid
  source 1..13: mol_type = other DNA
cgatctgaggtat

SEQ ID NO: 191 - DNA, 19 bp, synthetic construct
  misc_feature 1..19: note = Synthetic Construct
  misc_feature 4: note = locked nucleic acid
  misc_feature 11: note = locked nucleic acid
  misc_feature 18: note = locked nucleic acid
  source 1..19: mol_type = other DNA
aatccatttggaatatgta

SEQ ID NO: 192 - DNA, 23 bp, synthetic construct
  misc_feature 1..23: note = Synthetic Construct
  misc_feature 4: note = locked nucleic acid
  misc_feature 8: note = locked nucleic acid
  misc_feature 10: note = locked nucleic acid
  misc_feature 14: note = locked nucleic acid
  source 1..23: mol_type = other DNA
ccatatacagaataattataatg

SEQ ID NO: 193 - DNA, 13 bp, synthetic construct
  misc_feature 1..13: note = Synthetic Construct
  misc_feature 3..5: note = locked nucleic acid
  misc_feature 10..11: note = locked nucleic acid
  source 1..13: mol_type = other DNA
ctgtgtttgcggt

SEQ ID NO: 194 - DNA, 19 bp, synthetic construct
  misc_feature 1..19: note = Synthetic Construct
  misc_feature 4..5: note = locked nucleic acid
  misc_feature 15..16: note = locked nucleic acid
  source 1..19: mol_type = other DNA
tgaaatattaattaggtgt

SEQ ID NO: 195 - DNA, 19 bp, synthetic construct
  misc_feature 1..19: note = Synthetic Construct
  misc_feature 16: note = locked nucleic acid
  source 1..19: mol_type = other DNA
tttaaatccacatgtcgtt

SEQ ID NO: 196 - DNA, 13 bp, synthetic construct
  misc_feature 1..13: note = Synthetic Construct
  misc_feature 3: note = locked nucleic acid
  misc_feature 7..10: note = locked nucleic acid
  misc_feature 12: note = locked nucleic acid
  source 1..13: mol_type = other DNA
tgtgtcctcaaga

SEQ ID NO: 197 - DNA, 19 bp, synthetic construct
  misc_feature 1..19: note = Synthetic Construct
  misc_feature 5: note = locked nucleic acid
  misc_feature 7: note = locked nucleic acid
  misc_feature 11: note = locked nucleic acid
  misc_feature 18: note = locked nucleic acid
  source 1..19: mol_type = other DNA
caaacgatttcataatatt

SEQ ID NO: 198 - DNA, 18 bp, synthetic construct
  misc_feature 1..18: note = Synthetic Construct
  source 1..18: mol_type = other DNA
cagtgcagtttctctacg

SEQ ID NO: 199 - DNA, 13 bp, synthetic construct
  misc_feature 1..13: note = Synthetic Construct
  misc_feature 4: note = locked nucleic acid
  misc_feature 6: note = locked nucleic acid
  misc_feature 10: note = locked nucleic acid
  source 1..13: mol_type = other DNA
acacgccgcacag

SEQ ID NO: 200 - DNA, 18 bp, synthetic construct
  misc_feature 1..18: note = Synthetic Construct
  source 1..18: mol_type = other DNA
acacaagccaacgttaaa

SEQ ID NO: 201 - DNA, 19 bp, synthetic construct
  misc_feature 1..19: note = Synthetic Construct
  misc_feature 12: note = locked nucleic acid
  misc_feature 15: note = locked nucleic acid
  source 1..19: mol_type = other DNA
aattgctcatagcagtata

SEQ ID NO: 202 - DNA, 13 bp, synthetic construct
  misc_feature 1..13: note = Synthetic Construct
  misc_feature 4..6: note = locked nucleic acid
  misc_feature 9..10: note = locked nucleic acid
  source 1..13: mol_type = other DNA
atcctgaaccaac

SEQ ID NO: 203 - DNA, 18 bp, synthetic construct
  misc_feature 1..18: note = Synthetic Construct
  source 1..18: mol_type = other DNA
aagtgacagctcagatga

SEQ ID NO: 204 - DNA, 20 bp, synthetic construct
  misc_feature 1..20: note = Synthetic Construct
  misc_feature 6: note = locked nucleic acid
  misc_feature 15: note = locked nucleic acid
  source 1..20: mol_type = other DNA
ttacaatgtagtaatcagct

SEQ ID NO: 205 - DNA, 13 bp, synthetic construct
  misc_feature 1..13: note = Synthetic Construct
  misc_feature 3: note = locked nucleic acid
  misc_feature 5..6: note = locked nucleic acid
  misc_feature 9: note = locked nucleic acid
  source 1..13: mol_type = other DNA
cggtccaagcctt

SEQ ID NO: 206 - DNA, 22 bp, synthetic construct
  misc_feature 1..22: note = Synthetic Construct
  source 1..22: mol_type = other DNA
taacaccacagttcgtttatgt

SEQ ID NO: 207 - DNA, 21 bp, synthetic construct
  misc_feature 1..21: note = Synthetic Construct
  source 1..21: mol_type = other DNA
acaatattcactgtgcccata

SEQ ID NO: 208 - DNA, 13 bp, synthetic construct
  misc_feature 1..13: note = Synthetic Construct
  misc_feature 3: note = locked nucleic acid
  misc_feature 5..6: note = locked nucleic acid
  misc_feature 8: note = locked nucleic acid
  misc_feature 10..11: note = locked nucleic acid
  source 1..13: mol_type = other DNA
tgacctacgaacc

SEQ ID NO: 209 - DNA, 13 bp, synthetic construct
  misc_feature 1..13: note = Synthetic Construct
  misc_feature 4: note = locked nucleic acid
  misc_feature 6..7: note = locked nucleic acid
  misc_feature 9: note = locked nucleic acid
  misc_feature 11..12: note = locked nucleic acid
  source 1..13: mol_type = other DNA
cagtacagcaagt

SEQ ID NO: 210 - DNA, 19 bp, synthetic construct
  misc_feature 1..19: note = Synthetic Construct
  misc_feature 15: note = locked nucleic acid
  source 1..19: mol_type = other DNA
caagcattggagacaacta

SEQ ID NO: 211 - DNA, 18 bp, synthetic construct
  misc_feature 1..18: note = Synthetic Construct
  misc_feature 15: note = locked nucleic acid
  source 1..18: mol_type = other DNA
tatacctcagatcgttgc

SEQ ID NO: 212 - DNA, 13 bp, synthetic construct
  misc_feature 1..13: note = Synthetic Construct
  misc_feature 3: note = locked nucleic acid
  misc_feature 5..6: note = locked nucleic acid
  misc_feature 10: note = locked nucleic acid
  misc_feature 12: note = locked nucleic acid
  source 1..13: mol_type = other DNA
tccacgcactgta

SEQ ID NO: 213 - DNA, 18 bp, synthetic construct
  misc_feature 1..18: note = Synthetic Construct
  misc_feature 6: note = locked nucleic acid
  source 1..18: mol_type = other DNA
tgattttgcatttgcaga

SEQ ID NO: 214 - DNA, 18 bp, synthetic construct
  misc_feature 1..18: note = Synthetic Construct
  misc_feature 5: note = locked nucleic acid
  misc_feature 9: note = locked nucleic acid
  misc_feature 14: note = locked nucleic acid
  source 1..18: mol_type = other DNA
caaacacagtttacatat

SEQ ID NO: 215 - DNA, 13 bp, synthetic construct
  misc_feature 1..13: note = Synthetic Construct
  misc_feature 3..5: note = locked nucleic acid
  misc_feature 7..9: note = locked nucleic acid
  source 1..13: mol_type = other DNA
ttccctctctata

SEQ ID NO: 216 - DNA, 20 bp, synthetic construct
  misc_feature 1..20: note = Synthetic Construct
  misc_feature 4..5: note = locked nucleic acid
  misc_feature 9: note = locked nucleic acid
  misc_feature 18: note = locked nucleic acid
  source 1..20: mol_type = other DNA
gttcttatctaaaattagtg

SEQ ID NO: 217 - DNA, 21 bp, synthetic construct
  misc_feature 1..21: note = Synthetic Construct
  misc_feature 9: note = locked nucleic acid
  misc_feature 16: note = locked nucleic acid
  source 1..21: mol_type = other DNA
tttaactgtttgttctaatgt

SEQ ID NO: 218 - DNA, 13 bp, synthetic construct
  misc_feature 1..13: note = Synthetic Construct
  misc_feature 3..5: note = locked nucleic acid
  misc_feature 10..12: note = locked nucleic acid
  source 1..13: mol_type = other DNA
ttccatatacaga

SEQ ID NO: 219 - DNA, 13 bp, synthetic construct
  misc_feature 1..13: note = Synthetic Construct
  misc_feature 2: note = locked nucleic acid
  misc_feature 5: note = locked nucleic acid
  misc_feature 9..12: note = locked nucleic acid
  source 1..13: mol_type = other DNA
tctgtatatggaa

SEQ ID NO: 220 - DNA, 21 bp, synthetic construct
  misc_feature 1..21: note = Synthetic Construct
  misc_feature 14: note = locked nucleic acid
  misc_feature 20: note = locked nucleic acid
  source 1..21: mol_type = other DNA
aggtgtattatatgtcaaaga

SEQ ID NO: 221 - DNA, 20 bp, synthetic construct
  misc_feature 1..20: note = Synthetic Construct
  misc_feature 13..15: note = locked nucleic acid
  source 1..20: mol_type = other DNA
atattatgaaatcgtttgtt

SEQ ID NO: 222 - DNA, 13 bp, synthetic construct
  misc_feature 1..13: note = Synthetic Construct
  misc_feature 3: note = locked nucleic acid
  misc_feature 5: note = locked nucleic acid
  misc_feature 7..9: note = locked nucleic acid
  misc_feature 12: note = locked nucleic acid
  source 1..13: mol_type = other DNA
ttgtgtcctcaag

SEQ ID NO: 223 - DNA, 13 bp, synthetic construct
  misc_feature 1..13: note = Synthetic Construct
  misc_feature 3..4: note = locked nucleic acid
  misc_feature 9..11: note = locked nucleic acid
  source 1..13: mol_type = other DNA
cgacatgtggatt

SEQ ID NO: 224 - DNA, 18 bp, synthetic construct
  misc_feature 1..18: note = Synthetic Construct
  misc_feature 3..4: note = locked nucleic acid
  misc_feature 11: note = locked nucleic acid
  misc_feature 15: note = locked nucleic acid
  source 1..18: mol_type = other DNA
aggaatatgttttagatt

SEQ ID NO: 225 - DNA, 18 bp, synthetic construct
  misc_feature 1..18: note = Synthetic Construct
  misc_feature 16: note = locked nucleic acid
  source 1..18: mol_type = other DNA
atctgagctgtcacttaa

SEQ ID NO: 226 - DNA, 13 bp, synthetic construct
  misc_feature 1..13: note = Synthetic Construct
  misc_feature 3..6: note = locked nucleic acid
  misc_feature 8: note = locked nucleic acid
  misc_feature 10: note = locked nucleic acid
  source 1..13: mol_type = other DNA
tgacctatactgc

SEQ ID NO: 227 - DNA, 17 bp, synthetic construct
  misc_feature 1..17: note = Synthetic Construct
  source 1..17: mol_type = other DNA
gaggatgaaggcttgga

SEQ ID NO: 228 - DNA, 17 bp, synthetic construct
  misc_feature 1..17: note = Synthetic Construct
  misc_feature 6: note = locked nucleic acid
  misc_feature 14: note = locked nucleic acid
  source 1..17: mol_type = other DNA
tgacaacaggttacaat

SEQ ID NO: 229 - DNA, 23 bp, synthetic construct
  misc_feature 1..23: note = Synthetic Construct
  source 1..23: mol_type = other DNA
ccagatggacaagcacaaccagc

SEQ ID NO: 230 - DNA, 17 bp, synthetic construct
  misc_feature 1..17: note = Synthetic Construct
  misc_feature 6: note = locked nucleic acid
  source 1..17: mol_type = other DNA
tgtcaacagtacagcaa

SEQ ID NO: 231 - DNA, 18 bp, synthetic construct
  misc_feature 1..18: note = Synthetic Construct
  source 1..18: mol_type = other DNA
aggtagggcacacaatat

SEQ ID NO: 232 - DNA, 13 bp, synthetic construct
  misc_feature 1..13: note = Synthetic Construct
  misc_feature 3..4: note = locked nucleic acid
  misc_feature 7..10: note = locked nucleic acid
  source 1..13: mol_type = other DNA
accatacagcaac

SEQ ID NO: 233 - DNA, 17 bp, synthetic construct
  misc_feature 1..17: note = Synthetic Construct
  misc_feature 5: note = locked nucleic acid
  misc_feature 8: note = locked nucleic acid
  source 1..17: mol_type = other DNA
ctgaacgaccttacaaa

SEQ ID NO: 234 - DNA, 18 bp, synthetic construct
  misc_feature 1..18: note = Synthetic Construct
  misc_feature 11: note = locked nucleic acid
  misc_feature 15..16: note = locked nucleic acid
  source 1..18: mol_type = other DNA
atacacaattcaaacaaa

SEQ ID NO: 235 - DNA, 28 bp, synthetic construct
  misc_feature 1..28: note = Synthetic Construct
  source 1..28: mol_type = other DNA
tgatttgtgcaacgaggtagaagaaagc

SEQ ID NO: 236 - DNA, 13 bp, synthetic construct
  misc_feature 1..13: note = Synthetic Construct
  misc_feature 3: note = locked nucleic acid
  misc_feature 5..8: note = locked nucleic acid
  misc_feature 11: note = locked nucleic acid
  source 1..13: mol_type = other DNA
cgaggtagaagaa

SEQ ID NO: 237 - DNA, 16 bp, synthetic construct
  misc_feature 1..16: note = Synthetic Construct
  misc_feature 5: note = locked nucleic acid
  misc_feature 11: note = locked nucleic acid
  misc_feature 15: note = locked nucleic acid
  source 1..16: mol_type = other DNA
caaacaagaattacag

SEQ ID NO: 238 - DNA, 18 bp, synthetic construct
  misc_feature 1..18: note = Synthetic Construct
  misc_feature 4..5: note = locked nucleic acid
  misc_feature 7: note = locked nucleic acid
  misc_feature 14: note = locked nucleic acid
  source 1..18: mol_type = other DNA
ccttctctatatactata

SEQ ID NO: 239 - DNA, 15 bp, synthetic construct
  misc_feature 1..15: note = Synthetic Construct
  misc_feature 3..6: note = locked nucleic acid
  misc_feature 10..11: note = locked nucleic acid
  source 1..15: mol_type = other DNA
agtcatatacctcac

SEQ ID NO: 240 - DNA, 18 bp, synthetic construct
  misc_feature 1..18: note = Synthetic Construct
  misc_feature 4..5: note = locked nucleic acid
  misc_feature 13..14: note = locked nucleic acid
  source 1..18: mol_type = other DNA
attcaaaaataagtgaat

SEQ ID NO: 241 - DNA, 19 bp, synthetic construct
  misc_feature 1..19: note = Synthetic Construct
  misc_feature 13: note = locked nucleic acid
  source 1..19: mol_type = other DNA
taactgtttgttgcattgt

SEQ ID NO: 242 - DNA, 13 bp, synthetic construct
  misc_feature 1..13: note = Synthetic Construct
  misc_feature 3..5: note = locked nucleic acid
  misc_feature 10..12: note = locked nucleic acid
  source 1..13: mol_type = other DNA
tagtgtgtatgga

SEQ ID NO: 243 - DNA, 19 bp, synthetic construct
  misc_feature 1..19: note = Synthetic Construct
  misc_feature 8: note = locked nucleic acid
  misc_feature 10..11: note = locked nucleic acid
  misc_feature 16: note = locked nucleic acid
  source 1..19: mol_type = other DNA
tgtcatttattaattaggt

SEQ ID NO: 244 - DNA, 19 bp, synthetic construct
  misc_feature 1..19: note = Synthetic Construct
  misc_feature 10: note = locked nucleic acid
  misc_feature 14: note = locked nucleic acid
  source 1..19: mol_type = other DNA
ttcttctaaatgtctttgc

SEQ ID NO: 245 - DNA, 13 bp, synthetic construct
  misc_feature 1..13: note = Synthetic Construct
  misc_feature 3..4: note = locked nucleic acid
  misc_feature 10..12: note = locked nucleic acid
  source 1..13: mol_type = other DNA
tgtcaaaaaccgc

SEQ ID NO: 246 - DNA, 18 bp, synthetic construct
  misc_feature 1..18: note = Synthetic Construct
  misc_feature 13: note = locked nucleic acid
  source 1..18: mol_type = other DNA
cgattccataacatcggt

SEQ ID NO: 247 - DNA, 17 bp, synthetic construct
  misc_feature 1..17: note = Synthetic Construct
  source 1..17: mol_type = other DNA
tcggtttctctacgtgt

SEQ ID NO: 248 - DNA, 13 bp, synthetic construct
  misc_feature 1..13: note = Synthetic Construct
  misc_feature 3..6: note = locked nucleic acid
  misc_feature 9..10: note = locked nucleic acid
  source 1..13: mol_type = other DNA
cggtgtatgtcct

SEQ ID NO: 249 - DNA, 18 bp, synthetic construct
  misc_feature 1..18: note = Synthetic Construct
  misc_feature 7: note = locked nucleic acid
  misc_feature 9: note = locked nucleic acid
  misc_feature 17: note = locked nucleic acid
  source 1..18: mol_type = other DNA
catggagaaataactaca

SEQ ID NO: 250 - DNA, 18 bp, synthetic construct
  misc_feature 1..18: note = Synthetic Construct
  misc_feature 10: note = locked nucleic acid
  misc_feature 13: note = locked nucleic acid
  misc_feature 15: note = locked nucleic acid
  source 1..18: mol_type = other DNA
ctcataacagtataggtc

SEQ ID NO: 251 - DNA, 13 bp, synthetic construct
  misc_feature 1..13: note = Synthetic Construct
  misc_feature 3: note = locked nucleic acid
  misc_feature 6: note = locked nucleic acid
  misc_feature 8..9: note = locked nucleic acid
  misc_feature 11..12: note = locked nucleic acid
  source 1..13: mol_type = other DNA
tgcaagactatgt

SEQ ID NO: 252 - DNA, 17 bp, synthetic construct
  misc_feature 1..17: note = Synthetic Construct
  misc_feature 5: note = locked nucleic acid
  source 1..17: mol_type = other DNA
aattgtgtgacagctca

SEQ ID NO: 253 - DNA, 18 bp, synthetic construct
  misc_feature 1..18: note = Synthetic Construct
  source 1..18: mol_type = other DNA
taattggaggtgtctggt

SEQ ID NO: 254 - DNA, 13 bp, synthetic construct
  misc_feature 1..13: note = Synthetic Construct
  misc_feature 3..5: note = locked nucleic acid
  misc_feature 7: note = locked nucleic acid
  misc_feature 10..11: note = locked nucleic acid
  source 1..13: mol_type = other DNA
ttgcttgtccagc

SEQ ID NO: 255 - DNA, 19 bp, synthetic construct
  misc_feature 1..19: note = Synthetic Construct
  misc_feature 3: note = locked nucleic acid
  misc_feature 15: note = locked nucleic acid
  source 1..19: mol_type = other DNA
taatattgtaacgtcctgt

SEQ ID NO: 256 - DNA, 19 bp, synthetic construct
  misc_feature 1..19: note = Synthetic Construct
  misc_feature 3: note = locked nucleic acid
  misc_feature 5: note = locked nucleic acid
  misc_feature 11: note = locked nucleic acid
  misc_feature 16: note = locked nucleic acid
  source 1..19: mol_type = other DNA
ataaatcttccaatttacg

SEQ ID NO: 257 - DNA, 13 bp, synthetic construct
  misc_feature 1..13: note = Synthetic Construct
  misc_feature 3..4: note = locked nucleic acid
  misc_feature 6..7: note = locked nucleic acid
  misc_feature 12: note = locked nucleic acid
  source 1..13: mol_type = other DNA
cactacgtctgtg

SEQ ID NO: 258 - DNA, 17 bp, synthetic construct
  misc_feature 1..17: note = Synthetic Construct
  misc_feature 13: note = locked nucleic acid
  source 1..17: mol_type = other DNA
tgcatgatttgtgcaac

SEQ ID NO: 259 - DNA, 18 bp, synthetic construct
  misc_feature 1..18: note = Synthetic Construct
  misc_feature 5: note = locked nucleic acid
  misc_feature 14: note = locked nucleic acid
  source 1..18: mol_type = other DNA
cttgtttgcagtatacac

SEQ ID NO: 260 - DNA, 13 bp, synthetic construct
  misc_feature 1..13: note = Synthetic Construct
  misc_feature 5..6: note = locked nucleic acid
  misc_feature 8..10: note = locked nucleic acid
  misc_feature 12: note = locked nucleic acid
  source 1..13: mol_type = other DNA
aaagcatccatga

SEQ ID NO: 261 - DNA, 18 bp, synthetic construct
  misc_feature 1..18: note = Synthetic Construct
  source 1..18: mol_type = other DNA
cagcggagtgaggtatat

SEQ ID NO: 262 - DNA, 18 bp, synthetic construct
  misc_feature 1..18: note = Synthetic Construct
  misc_feature 5: note = locked nucleic acid
  misc_feature 8: note = locked nucleic acid
  misc_feature 10: note = locked nucleic acid
  misc_feature 15..16: note = locked nucleic acid
  source 1..18: mol_type = other DNA
aattttaaacatttcatg

SEQ ID NO: 263 - DNA, 13 bp, synthetic construct
  misc_feature 1..13: note = Synthetic Construct
  misc_feature 3: note = locked nucleic acid
  misc_feature 5: note = locked nucleic acid
  misc_feature 8: note = locked nucleic acid
  misc_feature 11..12: note = locked nucleic acid
  source 1..13: mol_type = other DNA
agagaaggccagc

SEQ ID NO: 264 - DNA, 21 bp, synthetic construct
  misc_feature 1..21: note = Synthetic Construct
  misc_feature 4: note = locked nucleic acid
  misc_feature 7: note = locked nucleic acid
  misc_feature 11: note = locked nucleic acid
  misc_feature 16..17: note = locked nucleic acid
  source 1..21: mol_type = other DNA
aatatagatggtatagatata

SEQ ID NO: 265 - DNA, 20 bp, synthetic construct
  misc_feature 1..20: note = Synthetic Construct
  misc_feature 5: note = locked nucleic acid
  misc_feature 8: note = locked nucleic acid
  misc_feature 10: note = locked nucleic acid
  misc_feature 17: note = locked nucleic acid
  source 1..20: mol_type = other DNA
aataaatgacataactgttt

SEQ ID NO: 266 - DNA, 13 bp, synthetic construct
  misc_feature 1..13: note = Synthetic Construct
  misc_feature 3..6: note = locked nucleic acid
  misc_feature 8: note = locked nucleic acid
  misc_feature 10: note = locked nucleic acid
  source 1..13: mol_type = other DNA
ttctccatacaca

SEQ ID NO: 267 - DNA, 18 bp, synthetic construct
  misc_feature 1..18: note = Synthetic Construct
  misc_feature 3: note = locked nucleic acid
  misc_feature 6: note = locked nucleic acid
  misc_feature 9: note = locked nucleic acid
  misc_feature 17: note = locked nucleic acid
  source 1..18: mol_type = other DNA
aattaggtgtattacatg

SEQ ID NO: 268 - DNA, 18 bp, synthetic construct
  misc_feature 1..18: note = Synthetic Construct
  misc_feature 4: note = locked nucleic acid
  misc_feature 10: note = locked nucleic acid
  misc_feature 14: note = locked nucleic acid
  source 1..18: mol_type = other DNA
aatcgttttttttcttct

SEQ ID NO: 269 - DNA, 14 bp, synthetic construct
  misc_feature 1..14: note = Synthetic Construct
  misc_feature 1..5: note = locked nucleic acid
  misc_feature 7: note = locked nucleic acid
  misc_feature 12: note = locked nucleic acid
  source 1..14: mol_type = other DNA
ccagttgaaaagca

SEQ ID NO: 270 - DNA, 17 bp, synthetic construct
  misc_feature 1..17: note = Synthetic Construct
  misc_feature 3: note = locked nucleic acid
  source 1..17: mol_type = other DNA
ccataacatcggtggac

SEQ ID NO: 271 - DNA, 17 bp, synthetic construct
  misc_feature 1..17: note = Synthetic Construct
  misc_feature 3: note = locked nucleic acid
  source 1..17: mol_type = other DNA
acacctcggtttctcta

SEQ ID NO: 272 - DNA, 13 bp, synthetic construct
  misc_feature 1..13: note = Synthetic Construct
  misc_feature 4: note = locked nucleic acid
  misc_feature 7..10: note = locked nucleic acid
  misc_feature 12: note = locked nucleic acid
  source 1..13: mol_type = other DNA
tgtatgtcctgtt

SEQ ID NO: 273 - DNA, 18 bp, synthetic construct
  misc_feature 1..18: note = Synthetic Construct
  misc_feature 13: note = locked nucleic acid
  source 1..18: mol_type = other DNA
tttagatttggaacccga

SEQ ID NO: 274 - DNA, 17 bp, synthetic construct
  misc_feature 1..17: note = Synthetic Construct
  misc_feature 13: note = locked nucleic acid
  source 1..17: mol_type = other DNA
tatcttcctcctcctct

SEQ ID NO: 275 - DNA, 13 bp, synthetic construct
  misc_feature 1..13: note = Synthetic Construct
  misc_feature 3..7: note = locked nucleic acid
  misc_feature 12: note = locked nucleic acid
  source 1..13: mol_type = other DNA
actgacctatact

SEQ ID NO: 276 - DNA, 17 bp, synthetic construct
  misc_feature 1..17: note = Synthetic Construct
  source 1..17: mol_type = other DNA
ctattgacggtccagct

SEQ ID NO: 277 - DNA, 18 bp, synthetic construct
  misc_feature 1..18: note = Synthetic Construct
  misc_feature 7: note = locked nucleic acid
  misc_feature 10: note = locked nucleic acid
  source 1..18: mol_type = other DNA
catttacaacaggacgtt

SEQ ID NO: 278 - DNA, 12 bp, synthetic construct
  misc_feature 1..12: note = Synthetic Construct
  misc_feature 4..8: note = locked nucleic acid
  misc_feature 10: note = locked nucleic acid
  source 1..12: mol_type = other DNA
ccagacacctcc

SEQ ID NO: 279 - DNA, 17 bp, synthetic construct
  misc_feature 1..17: note = Synthetic Construct
  source 1..17: mol_type = other DNA
tgaggcgacactacgtc

SEQ ID NO: 280 - DNA, 23 bp, synthetic construct
  misc_feature 1..23: note = Synthetic Construct
  source 1..23: mol_type = other DNA
gtgcccattaataaatcttccaa

SEQ ID NO: 281 - DNA, 13 bp, synthetic construct
  misc_feature 1..13: note = Synthetic Construct
  misc_feature 2: note = locked nucleic acid
  misc_feature 5..6: note = locked nucleic acid
  misc_feature 9..10: note = locked nucleic acid
  source 1..13: mol_type = other DNA
agagcacacacat

SEQ ID NO: 282 - DNA, 17 bp, synthetic construct
  misc_feature 1..17: note = Synthetic Construct
  misc_feature 5: note = locked nucleic acid
  misc_feature 8: note = locked nucleic acid
  source 1..17: mol_type = other DNA
ctgaacgaccttacaaa

SEQ ID NO: 283 - DNA, 18 bp, synthetic construct
  misc_feature 1..18: note = Synthetic Construct
  misc_feature 11: note = locked nucleic acid
  misc_feature 15..16: note = locked nucleic acid
  source 1..18: mol_type = other DNA
atacacaattcaaacaaa

SEQ ID NO: 284 - DNA, 17 bp, synthetic construct
  misc_feature 1..17: note = Synthetic Construct
  source 1..17: mol_type = other DNA
cgctttgacgatccaaa

SEQ ID NO: 285 - DNA, 18 bp, synthetic construct
  misc_feature 1..18: note = Synthetic Construct
  misc_feature 4: note = locked nucleic acid
  misc_feature 8: note = locked nucleic acid
  misc_feature 14: note = locked nucleic acid
  source 1..18: mol_type = other DNA
tcttgtagtgatgtattc

SEQ ID NO: 286 - DNA, 12 bp, synthetic construct
  misc_feature 1..12: note = Synthetic Construct
  misc_feature 3..4: note = locked nucleic acid
  misc_feature 6..8: note = locked nucleic acid
  misc_feature 10: note = locked nucleic acid
  source 1..12: mol_type = other DNA
agctaccagatt

SEQ ID NO: 287 - DNA, 18 bp, synthetic construct
  misc_feature 1..18: note = Synthetic Construct
  misc_feature 9: note = locked nucleic acid
  source 1..18: mol_type = other DNA
cgtatctattgcctgtgt

SEQ ID NO: 288 - DNA, 20 bp, synthetic construct
  misc_feature 1..20: note = Synthetic Construct
  misc_feature 8..10: note = locked nucleic acid
  misc_feature 15: note = locked nucleic acid
  source 1..20: mol_type = other DNA
cactatacataaatctttaa

SEQ ID NO: 289 - DNA, 29 bp, synthetic construct
  misc_feature 1..29: note = Synthetic Construct
  source 1..29: mol_type = other DNA
agcaacattggaacgcacagaggtatatc

SEQ ID NO: 290 - DNA, 17 bp, synthetic construct
  misc_feature 1..17: note = Synthetic Construct
  misc_feature 8: note = locked nucleic acid
  misc_feature 10: note = locked nucleic acid
  misc_feature 14: note = locked nucleic acid
  source 1..17: mol_type = other DNA
atagagactgtatagca

SEQ ID NO: 291 - DNA, 20 bp, synthetic construct
  misc_feature 1..20: note = Synthetic Construct
  misc_feature 5: note = locked nucleic acid
  misc_feature 12..14: note = locked nucleic acid
  source 1..20: mol_type = other DNA
atatcttaattctctaattc

SEQ ID NO: 292 - DNA, 14 bp, synthetic construct
  misc_feature 1..14: note = Synthetic Construct
  misc_feature 3..4: note = locked nucleic acid
  misc_feature 9..12: note = locked nucleic acid
  source 1..14: mol_type = other DNA
tacatttatggcat

SEQ ID NO: 293 - DNA, 18 bp, synthetic construct
  misc_feature 1..18: note = Synthetic Construct
  misc_feature 5: note = locked nucleic acid
  misc_feature 10..11: note = locked nucleic acid
  misc_feature 16: note = locked nucleic acid
  source 1..18: mol_type = other DNA
tattcaaactctgtatat

SEQ ID NO: 294 - DNA, 19 bp, synthetic construct
  misc_feature 1..19: note = Synthetic Construct
  misc_feature 4..5: note = locked nucleic acid
  misc_feature 12..13: note = locked nucleic acid
  source 1..19: mol_type = other DNA
caccttattaacaaattat

SEQ ID NO: 295 - DNA, 13 bp, synthetic construct
  misc_feature 1..13: note = Synthetic Construct
  misc_feature 3..4: note = locked nucleic acid
  misc_feature 8..9: note = locked nucleic acid
  misc_feature 11: note = locked nucleic acid
  source 1..13: mol_type = other DNA
tccagtgtctctc

SEQ ID NO: 296 - DNA, 17 bp, synthetic construct
  misc_feature 1..17: note = Synthetic Construct
  misc_feature 6: note = locked nucleic acid
  misc_feature 10: note = locked nucleic acid
  source 1..17: mol_type = other DNA
ccagaaaccattgaacc

SEQ ID NO: 297 - DNA, 18 bp, synthetic construct
  misc_feature 1..18: note = Synthetic Construct
  misc_feature 15: note = locked nucleic acid
  source 1..18: mol_type = other DNA
agctatgctgtgaaatct

SEQ ID NO: 298 - DNA, 12 bp, synthetic construct
  misc_feature 1..12: note = Synthetic Construct
  misc_feature 3..4: note = locked nucleic acid
  misc_feature 6..8: note = locked nucleic acid
  misc_feature 10: note = locked nucleic acid
  source 1..12: mol_type = other DNA
cgtagacacctt

SEQ ID NO: 299 - DNA, 17 bp, synthetic construct
  misc_feature 1..17: note = Synthetic Construct
  misc_feature 14: note = locked nucleic acid
  source 1..17: mol_type = other DNA
cgagggcagtgtaatac

SEQ ID NO: 300 - DNA, 17 bp, synthetic construct
  misc_feature 1..17: note = Synthetic Construct
  misc_feature 8: note = locked nucleic acid
  source 1..17: mol_type = other DNA
cttgtgtttccctacgt

SEQ ID NO: 301 - DNA, 13 bp, synthetic construct
  misc_feature 1..13: note = Synthetic Construct
  misc_feature 3..4: note = locked nucleic acid
  misc_feature 6..7: note = locked nucleic acid
  misc_feature 10..11: note = locked nucleic acid
  source 1..13: mol_type = other DNA
cctggtcacaaca

SEQ ID NO: 302 - DNA, 22 bp, synthetic construct
  misc_feature 1..22: note = Synthetic Construct
  source 1..22: mol_type = other DNA
tgaccaggcacggcaagaaaga

SEQ ID NO: 303 - DNA, 19 bp, synthetic construct
  misc_feature 1..19: note = Synthetic Construct
  misc_feature 16: note = locked nucleic acid
  source 1..19: mol_type = other DNA
aacactgcaagaaattgta

SEQ ID NO: 304 - DNA, 17 bp, synthetic construct
  misc_feature 1..17: note = Synthetic Construct
  misc_feature 12: note = locked nucleic acid
  source 1..17: mol_type = other DNA
ctcgtaacacaacaggt

SEQ ID NO: 305 - DNA, 13 bp, synthetic construct
  misc_feature 1..13: note = Synthetic Construct
  misc_feature 6..7: note = locked nucleic acid
  misc_feature 9: note = locked nucleic acid
  misc_feature 11..12: note = locked nucleic acid
  source 1..13: mol_type = other DNA
tggaacctcagaa

SEQ ID NO: 306 - DNA, 18 bp, synthetic construct
  misc_feature 1..18: note = Synthetic Construct
  misc_feature 11: note = locked nucleic acid
  source 1..18: mol_type = other DNA
caattaagcgagtcagag

SEQ ID NO: 307 - DNA, 17 bp, synthetic construct
  misc_feature 1..17: note = Synthetic Construct
  source 1..17: mol_type = other DNA
gtcgggctggtagttgt

SEQ ID NO: 308 - DNA, 13 bp, synthetic construct
  misc_feature 1..13: note = Synthetic Construct
  misc_feature 3..6: note = locked nucleic acid
  misc_feature 10: note = locked nucleic acid
  misc_feature 12: note = locked nucleic acid
  source 1..13: mol_type = other DNA
cgatgaagcagat

SEQ ID NO: 309 - DNA, 18 bp, synthetic construct
  misc_feature 1..18: note = Synthetic Construct
  misc_feature 9..10: note = locked nucleic acid
  misc_feature 16: note = locked nucleic acid
  source 1..18: mol_type = other DNA
aattttgtgtgtatgttg

SEQ ID NO: 310 - DNA, 17 bp, synthetic construct
  misc_feature 1..17: note = Synthetic Construct
  misc_feature 4: note = locked nucleic acid
  misc_feature 11: note = locked nucleic acid
  source 1..17: mol_type = other DNA
ctgctgtagtgttctaa

SEQ ID NO: 311 - DNA, 13 bp, synthetic construct
  misc_feature 1..13: note = Synthetic Construct
  misc_feature 3..5: note = locked nucleic acid
  misc_feature 7..8: note = locked nucleic acid
  misc_feature 10: note = locked nucleic acid
  source 1..13: mol_type = other DNA
acggcagaattga

SEQ ID NO: 312 - DNA, 18 bp, synthetic construct
  misc_feature 1..18: note = Synthetic Construct
  misc_feature 10: note = locked nucleic acid
  source 1..18: mol_type = other DNA
cctacaagctaccagatt

SEQ ID NO: 313 - DNA, 18 bp, synthetic construct
  misc_feature 1..18: note = Synthetic Construct
  misc_feature 17: note = locked nucleic acid
  source 1..18: mol_type = other DNA
tgcaatatacacaggcaa

SEQ ID NO: 314 - DNA, 13 bp, synthetic construct
  misc_feature 1..13: note = Synthetic Construct
  misc_feature 3: note = locked nucleic acid
  misc_feature 6..7: note = locked nucleic acid
  misc_feature 9..11: note = locked nucleic acid
  source 1..13: mol_type = other DNA
cactacaagacgt

SEQ ID NO: 315 - DNA, 17 bp, synthetic construct
  misc_feature 1..17: note = Synthetic Construct
  source 1..17: mol_type = other DNA
aacattggaacgcacag

SEQ ID NO: 316 - DNA, 23 bp, synthetic construct
  misc_feature 1..23: note = Synthetic Construct
  misc_feature 17: note = locked nucleic acid
  source 1..23: mol_type = other DNA
tatgctatacagtctctatacac

SEQ ID NO: 317 - DNA, 18 bp, synthetic construct
  misc_feature 1..18: note = Synthetic Construct
  misc_feature 3..5: note = locked nucleic acid
  misc_feature 8..9: note = locked nucleic acid
  misc_feature 16: note = locked nucleic acid
  source 1..18: mol_type = other DNA
aggtatatcaatttgctt

SEQ ID NO: 318 - DNA, 20 bp, synthetic construct
  misc_feature 1..20: note = Synthetic Construct
  misc_feature 4: note = locked nucleic acid
  misc_feature 10: note = locked nucleic acid
  misc_feature 19: note = locked nucleic acid
  source 1..20: mol_type = other DNA
catgccataaatgtatagac

SEQ ID NO: 319 - DNA, 18 bp, synthetic construct
  misc_feature 1..18: note = Synthetic Construct
  misc_feature 3: note = locked nucleic acid
  misc_feature 6: note = locked nucleic acid
  misc_feature 12: note = locked nucleic acid
  source 1..18: mol_type = other DNA
ccatatacagagtttgaa

SEQ ID NO: 320 - DNA, 14 bp, synthetic construct
  misc_feature 1..14: note = Synthetic Construct
  misc_feature 2..5: note = locked nucleic acid
  misc_feature 11..12: note = locked nucleic acid
  source 1..14: mol_type = other DNA
tccagaattagaga

SEQ ID NO: 321 - DNA, 20 bp, synthetic construct
  misc_feature 1..20: note = Synthetic Construct
  misc_feature 8: note = locked nucleic acid
  misc_feature 12: note = locked nucleic acid
  misc_feature 15: note = locked nucleic acid
  source 1..20: mol_type = other DNA
aataactaatacagagttgt

SEQ ID NO: 322 - DNA, 17 bp, synthetic construct
  misc_feature 1..17: note = Synthetic Construct
  misc_feature 14: note = locked nucleic acid
  source 1..17: mol_type = other DNA
tgtctacgtttttctgc

SEQ ID NO: 323 - DNA, 13 bp, synthetic construct
  misc_feature 1..13: note = Synthetic Construct
  misc_feature 3..5: note = locked nucleic acid
  misc_feature 8..10: note = locked nucleic acid
  source 1..13: mol_type = other DNA
aaccattgaaccc

SEQ ID NO: 324 - DNA, 24 bp, synthetic construct
  misc_feature 1..24: note = Synthetic Construct
  source 1..24: mol_type = other DNA
ttgttaataaggtgcctgcggtgc

SEQ ID NO: 325 - DNA, 18 bp, synthetic construct
  misc_feature 1..18: note = Synthetic Construct
  misc_feature 8: note = locked nucleic acid
  misc_feature 10: note = locked nucleic acid
  source 1..18: mol_type = other DNA
ttaaggacaaacgaagat

SEQ ID NO: 326 - DNA, 17 bp, synthetic construct
  misc_feature 1..17: note = Synthetic Construct
  source 1..17: mol_type = other DNA
aagtctttcttgccgtg

SEQ ID NO: 327 - DNA, 26 bp, synthetic construct
  misc_feature 1..26: note = Synthetic Construct
  source 1..26: mol_type = other DNA
tggacagtaccgagggcagtgtaata

SEQ ID NO: 328 - DNA, 22 bp, synthetic construct
  misc_feature 1..22: note = Synthetic Construct
  source 1..22: mol_type = other DNA
tagctggacagtaccgagggca

SEQ ID NO: 329 - DNA, 20 bp, synthetic construct
  misc_feature 1..20: note = Synthetic Construct
  misc_feature 6: note = locked nucleic acid
  misc_feature 13: note = locked nucleic acid
  source 1..20: mol_type = other DNA
tcagaatgaattagatcctg

SEQ ID NO: 330 - DNA, 18 bp, synthetic construct
  misc_feature 1..18: note = Synthetic Construct
  source 1..18: mol_type = other DNA
tgcttcatcgttttcctc

SEQ ID NO: 331 - DNA, 13 bp, synthetic construct
  misc_feature 1..13: note = Synthetic Construct
  misc_feature 4..7: note = locked nucleic acid
  misc_feature 12: note = locked nucleic acid
  source 1..13: mol_type = other DNA
tgacctgttgtgt

SEQ ID NO: 332 - DNA, 18 bp, synthetic construct
  misc_feature 1..18: note = Synthetic Construct
  misc_feature 16: note = locked nucleic acid
  source 1..18: mol_type = other DNA
tagtcatgcacaactacc

SEQ ID NO: 333 - DNA, 19 bp, synthetic construct
  misc_feature 1..19: note = Synthetic Construct
  misc_feature 17: note = locked nucleic acid
  source 1..19: mol_type = other DNA
tcacacttacaacatacac

SEQ ID NO: 334 - DNA, 12 bp, synthetic construct
  misc_feature 1..12: note = Synthetic Construct
  misc_feature 5: note = locked nucleic acid
  misc_feature 7..8: note = locked nucleic acid
  source 1..12: mol_type = other DNA
ccgacgagccga

SEQ ID NO: 335 - DNA, 18 bp, synthetic construct
  misc_feature 1..18: note = Synthetic Construct
  source 1..18: mol_type = other DNA
cggcagaattgagcttac

SEQ ID NO: 336 - DNA, 18 bp, synthetic construct
  misc_feature 1..18: note = Synthetic Construct
  source 1..18: mol_type = other DNA
cggcagaattgagcttac

SEQ ID NO: 337 - DNA, 19 bp, synthetic construct
  misc_feature 1..19: note = Synthetic Construct
  source 1..19: mol_type = other DNA
ggacacacaaaggacaagg

SEQ ID NO: 338 - DNA, 18 bp, synthetic construct
  misc_feature 1..18: note = Synthetic Construct
  source 1..18: mol_type = other DNA
ggacacacaaaggacaag

SEQ ID NO: 339 - DNA, 13 bp, synthetic construct
  misc_feature 1..13: note = Synthetic Construct
  misc_feature 9: note = locked nucleic acid
  misc_feature 11..12: note = locked nucleic acid
  source 1..13: mol_type = other DNA
tcggcagaggacc

SEQ ID NO: 340 - DNA, 13 bp, synthetic construct
  misc_feature 1..13: note = Synthetic Construct
  misc_feature 6: note = locked nucleic acid
  misc_feature 9: note = locked nucleic acid
  misc_feature 11..12: note = locked nucleic acid
  source 1..13: mol_type = other DNA
tcggcagaggacc

SEQ ID NO: 341 - DNA, 16 bp, synthetic construct
  misc_feature 1..16: note = Synthetic Construct
  source 1..16: mol_type = other DNA
gggagaccgaagtgaa

SEQ ID NO: 342 - DNA, 16 bp, synthetic construct
  misc_feature 1..16: note = Synthetic Construct
  source 1..16: mol_type = other DNA
tccacttacctctggc

SEQ ID NO: 343 - DNA, 13 bp, synthetic construct
  misc_feature 1..13: note = Synthetic Construct
  misc_feature 3: note = locked nucleic acid
  misc_feature 6: note = locked nucleic acid
  misc_feature 8..10: note = locked nucleic acid
  source 1..13: mol_type = other DNA
ctggaccaacccg

SEQ ID NO: 344 - DNA, 17 bp, synthetic construct
  misc_feature 1..17: note = Synthetic Construct
  source 1..17: mol_type = other DNA
ctcggacagctcctaag

SEQ ID NO: 345 - DNA, 16 bp, synthetic construct
  misc_feature 1..16: note = Synthetic Construct
  misc_feature 9: note = locked nucleic acid
  source 1..16: mol_type = other DNA
acccttctacggactc

SEQ ID NO: 346 - DNA, 13 bp, synthetic construct
  misc_feature 1..13: note = Synthetic Construct
  misc_feature 3: note = locked nucleic acid
  misc_feature 9..10: note = locked nucleic acid
  misc_feature 12: note = locked nucleic acid
  source 1..13: mol_type = other DNA
cgcccagtcctac

SEQ ID NO: 347 - DNA, 17 bp, synthetic construct
  misc_feature 1..17: note = Synthetic Construct
  misc_feature 13: note = locked nucleic acid
  source 1..17: mol_type = other DNA
tctcttagagagtggct

SEQ ID NO: 348 - DNA, 18 bp, synthetic construct
  misc_feature 1..18: note = Synthetic Construct
  misc_feature 7: note = locked nucleic acid
  misc_feature 11: note = locked nucleic acid
  misc_feature 16: note = locked nucleic acid
  source 1..18: mol_type = other DNA
ttcttctatgtagacaga

SEQ ID NO: 349 - DNA, 13 bp, synthetic construct
  misc_feature 1..13: note = Synthetic Construct
  misc_feature 3..4: note = locked nucleic acid
  misc_feature 8..11: note = locked nucleic acid
  source 1..13: mol_type = other DNA
cgcattagagacc

SEQ ID NO: 350 - DNA, 18 bp, synthetic construct
  misc_feature 1..18: note = Synthetic Construct
  misc_feature 8: note = locked nucleic acid
  misc_feature 10: note = locked nucleic acid
  misc_feature 13: note = locked nucleic acid
  source 1..18: mol_type = other DNA
tgcctacattctatcttg

SEQ ID NO: 351 - DNA, 17 bp, synthetic construct
  misc_feature 1..17: note = Synthetic Construct
  source 1..17: mol_type = other DNA
acgggtttccaagacta

SEQ ID NO: 352 - DNA, 13 bp, synthetic construct
  misc_feature 1..13: note = Synthetic Construct
  misc_feature 3..5: note = locked nucleic acid
  misc_feature 9..10: note = locked nucleic acid
  misc_feature 12: note = locked nucleic acid
  source 1..13: mol_type = other DNA
tatgtttgtcccc

SEQ ID NO: 353 - DNA, 18 bp, synthetic construct
  misc_feature 1..18: note = Synthetic Construct
  misc_feature 12: note = locked nucleic acid
  source 1..18: mol_type = other DNA
cactctcagtaattccct

SEQ ID NO: 354 - DNA, 19 bp, synthetic construct
  misc_feature 1..19: note = Synthetic Construct
  misc_feature 7: note = locked nucleic acid
  misc_feature 9: note = locked nucleic acid
  misc_feature 17: note = locked nucleic acid
  source 1..19: mol_type = other DNA
caaagattgttagtggaat

SEQ ID NO: 355 - DNA, 13 bp, synthetic construct
  misc_feature 1..13: note = Synthetic Construct
  misc_feature 4: note = locked nucleic acid
  misc_feature 7: note = locked nucleic acid
  misc_feature 9..10: note = locked nucleic acid
  misc_feature 12: note = locked nucleic acid
  source 1..13: mol_type = other DNA
tccctaccaggaa

SEQ ID NO: 356 - DNA, 17 bp, synthetic construct
  misc_feature 1..17: note = Synthetic Construct
  source 1..17: mol_type = other DNA
ccgctaggatatgacgt

SEQ ID NO: 357 - DNA, 18 bp, synthetic construct
  misc_feature 1..18: note = Synthetic Construct
  misc_feature 10: note = locked nucleic acid
  misc_feature 15..17: note = locked nucleic acid
  source 1..18: mol_type = other DNA
ttacaatataattagcca

SEQ ID NO: 358 - DNA, 26 bp, synthetic construct
  misc_feature 1..26: note = Synthetic Construct
  source 1..26: mol_type = other DNA
acctctagcatctgctatgcgaatgc

SEQ ID NO: 359 - DNA, 16 bp, synthetic construct
  misc_feature 1..16: note = Synthetic Construct
  source 1..16: mol_type = other DNA
gcttacccctccacaa

SEQ ID NO: 360 - DNA, 16 bp, synthetic construct
  misc_feature 1..16: note = Synthetic Construct
  source 1..16: mol_type = other DNA
ggcaccgttagtgttg

SEQ ID NO: 361 - DNA, 21 bp, synthetic construct
  misc_feature 1..21: note = Synthetic Construct
  source 1..21: mol_type = other DNA
tacccctcctacccctctgcc

SEQ ID NO: 362 - DNA, 17 bp, synthetic construct
  misc_feature 1..17: note = Synthetic Construct
  source 1..17: mol_type = other DNA
taccgaacttcaaccca

SEQ ID NO: 363 - DNA, 18 bp, synthetic construct
  misc_feature 1..18: note = Synthetic Construct
  misc_feature 4: note = locked nucleic acid
  source 1..18: mol_type = other DNA
ttgatgagtaagagggtg

SEQ ID NO: 364 - DNA, 13 bp, synthetic construct
  misc_feature 1..13: note = Synthetic Construct
  misc_feature 3: note = locked nucleic acid
  misc_feature 8: note = locked nucleic acid
  misc_feature 10..12: note = locked nucleic acid
  source 1..13: mol_type = other DNA
ccatcaccaccac

SEQ ID NO: 365 - DNA, 13 bp, synthetic construct
  misc_feature 1..13: note = Synthetic Construct
  misc_feature 3..5: note = locked nucleic acid
  misc_feature 8: note = locked nucleic acid
  source 1..13: mol_type = other DNA
tgccagaccaatc

SEQ ID NO: 366 - DNA, 16 bp, synthetic construct
  misc_feature 1..16: note = Synthetic Construct
  misc_feature 10: note = locked nucleic acid
  source 1..16: mol_type = other DNA
agcaccccaaatgatc

SEQ ID NO: 367 - DNA, 17 bp, synthetic construct
  misc_feature 1..17: note = Synthetic Construct
  misc_feature 7: note = locked nucleic acid
  source 1..17: mol_type = other DNA
taatggcataggtggaa

SEQ ID NO: 368 - DNA, 19 bp, synthetic construct
  misc_feature 1..19: note = Synthetic Construct
  source 1..19: mol_type = other DNA
tccagaaccacggtccccg

SEQ ID NO: 369 - DNA, 19 bp, synthetic construct
  misc_feature 1..19: note = Synthetic Construct
  misc_feature 16: note = locked nucleic acid
  source 1..19: mol_type = other DNA
atcaacgaccaacaattac

SEQ ID NO: 370 - DNA, 18 bp, synthetic construct
  misc_feature 1..18: note = Synthetic Construct
  misc_feature 17: note = locked nucleic acid
  source 1..18: mol_type = other DNA
ttgagtcttagagggttg

SEQ ID NO: 371 - DNA, 13 bp, synthetic construct
  misc_feature 1..13: note = Synthetic Construct
  misc_feature 3..4: note = locked nucleic acid
  misc_feature 7: note = locked nucleic acid
  misc_feature 10: note = locked nucleic acid
  misc_feature 12: note = locked nucleic acid
  misc_feature 13: note = locked nucleic acid
  source 1..13: mol_type = other DNA
cccgagggtagat

SEQ ID NO: 372 - DNA, 15 bp, synthetic construct
  misc_feature 1..15: note = Synthetic Construct
  source 1..15: mol_type = other DNA
ttggagaccagagcc

SEQ ID NO: 373 - DNA, 17 bp, synthetic construct
  misc_feature 1..17: note = Synthetic Construct
  misc_feature 16: note = locked nucleic acid
  source 1..17: mol_type = other DNA
ttgtccctgatgaagac

SEQ ID NO: 374 - DNA, 13 bp, synthetic construct
  misc_feature 1..13: note = Synthetic Construct
  misc_feature 3..5: note = locked nucleic acid
  misc_feature 8..9: note = locked nucleic acid
  misc_feature 12: note = locked nucleic acid
  source 1..13: mol_type = other DNA
gcctgaactaagt

SEQ ID NO: 375 - DNA, 16 bp, synthetic construct
  misc_feature 1..16: note = Synthetic Construct
  source 1..16: mol_type = other DNA
actcaccaactcctgg

SEQ ID NO: 376 - DNA, 19 bp, synthetic construct
  misc_feature 1..19: note = Synthetic Construct
  misc_feature 12: note = locked nucleic acid
  source 1..19: mol_type = other DNA
ttcatgtattggtgaaacg

SEQ ID NO: 377 - DNA, 21 bp, synthetic construct
  misc_feature 1..21: note = Synthetic Construct
  source 1..21: mol_type = other DNA
caatgccgcccccgtttgtag

SEQ ID NO: 378 - DNA, 17 bp, synthetic construct
  misc_feature 1..17: note = Synthetic Construct
  misc_feature 13: note = locked nucleic acid
  source 1..17: mol_type = other DNA
cggagtcccataatagc

SEQ ID NO: 379 - DNA, 17 bp, synthetic construct
  misc_feature 1..17: note = Synthetic Construct
  source 1..17: mol_type = other DNA
gtctgcggggtctatag

SEQ ID NO: 380 - DNA, 13 bp, synthetic construct
  misc_feature 1..13: note = Synthetic Construct
  misc_feature 3..4: note = locked nucleic acid
  misc_feature 6..8: note = locked nucleic acid
  source 1..13: mol_type = other DNA
cagaggctcccat

SEQ ID NO: 381 - DNA, 18 bp, synthetic construct
  misc_feature 1..18: note = Synthetic Construct
  misc_feature 9: note = locked nucleic acid
  misc_feature 14: note = locked nucleic acid
  source 1..18: mol_type = other DNA
aaagttgggattacattt

SEQ ID NO: 382 - DNA, 17 bp, synthetic construct
  misc_feature 1..17: note = Synthetic Construct
  misc_feature 14: note = locked nucleic acid
  source 1..17: mol_type = other DNA
ggcgaggtcttttactg

SEQ ID NO: 383 - DNA, 30 bp, synthetic construct
  misc_feature 1..30: note = Synthetic Construct
  source 1..30: mol_type = other DNA
tgagacaacagaatctcctagctcagatga

SEQ ID NO: 384 - DNA, 19 bp, synthetic construct
  misc_feature 1..19: note = Synthetic Construct
  source 1..19: mol_type = other DNA
taggcccacttaacactac

SEQ ID NO: 385 - DNA, 18 bp, synthetic construct
  misc_feature 1..18: note = Synthetic Construct
  source 1..18: mol_type = other DNA
ggaggcccttagacttac

SEQ ID NO: 386 - DNA, 27 bp, synthetic construct
  misc_feature 1..27: note = Synthetic Construct
  source 1..27: mol_type = other DNA
cgcctctccattcatcatgtaacccac

SEQ ID NO: 387 - DNA, 21 bp, synthetic construct
  misc_feature 1..21: note = Synthetic Construct
  source 1..21: mol_type = other DNA
atccctaggataataccacac

SEQ ID NO: 388 - DNA, 17 bp, synthetic construct
  misc_feature 1..17: note = Synthetic Construct
  source 1..17: mol_type = other DNA
cacgtaaagccacaagc

SEQ ID NO: 389 - DNA, 27 bp, synthetic construct
  misc_feature 1..27: note = Synthetic Construct
  source 1..27: mol_type = other DNA
agcagtgtagtcctgtcaatctcctga

SEQ ID NO: 390 - DNA, 16 bp, synthetic construct
  misc_feature 1..16: note = Synthetic Construct
  misc_feature 13: note = locked nucleic acid
  source 1..16: mol_type = other DNA
ctcctaagaaggcacc

SEQ ID NO: 391 - DNA, 17 bp, synthetic construct
  misc_feature 1..17: note = Synthetic Construct
  source 1..17: mol_type = other DNA
ctcctcttcttgctgga

SEQ ID NO: 392 - DNA, 13 bp, synthetic construct
  misc_feature 1..13: note = Synthetic Construct
  misc_feature 3..5: note = locked nucleic acid
  misc_feature 8: note = locked nucleic acid
  misc_feature 12: note = locked nucleic acid
  source 1..13: mol_type = other DNA
caagaacccagac

SEQ ID NO: 393 - DNA, 18 bp, synthetic construct
  misc_feature 1..18: note = Synthetic Construct
  misc_feature 4: note = locked nucleic acid
  misc_feature 11: note = locked nucleic acid
  misc_feature 16: note = locked nucleic acid
  source 1..18: mol_type = other DNA
attagagaccactttgag

SEQ ID NO: 394 - DNA, 19 bp, synthetic construct
  misc_feature 1..19: note = Synthetic Construct
  misc_feature 7: note = locked nucleic acid
  misc_feature 17: note = locked nucleic acid
  source 1..19: mol_type = other DNA
ttagtcttcatcctcttct

SEQ ID NO: 395 - DNA, 13 bp, synthetic construct
  misc_feature 1..13: note = Synthetic Construct
  misc_feature 3: note = locked nucleic acid
  misc_feature 5: note = locked nucleic acid
  misc_feature 8..11: note = locked nucleic acid
  source 1..13: mol_type = other DNA
cgccaatctgtct

SEQ ID NO: 396 - DNA, 19 bp, synthetic construct
  misc_feature 1..19: note = Synthetic Construct
  misc_feature 16: note = locked nucleic acid
  source 1..19: mol_type = other DNA
tctaattgttgacacggat

SEQ ID NO: 397 - DNA, 17 bp, synthetic construct
  misc_feature 1..17: note = Synthetic Construct
  misc_feature 6: note = locked nucleic acid
  source 1..17: mol_type = other DNA
tgtctgacagttgttcc

SEQ ID NO: 398 - DNA, 29 bp, synthetic construct
  misc_feature 1..29: note = Synthetic Construct
  source 1..29: mol_type = other DNA
cttggaaacccgtcactctcagtaattcc

SEQ ID NO: 399 - DNA, 19 bp, synthetic construct
  misc_feature 1..19: note = Synthetic Construct
  source 1..19: mol_type = other DNA
tcacctcttgatagggatc

SEQ ID NO: 400 - DNA, 18 bp, synthetic construct
  misc_feature 1..18: note = Synthetic Construct
  misc_feature 17: note = locked nucleic acid
  source 1..18: mol_type = other DNA
attagccatccaaagcat

SEQ ID NO: 401 - DNA, 22 bp, synthetic construct
  misc_feature 1..22: note = Synthetic Construct
  source 1..22: mol_type = other DNA
cgggcatggacctctagcatct

SEQ ID NO: 402 - DNA, 18 bp, synthetic construct
  misc_feature 1..18: note = Synthetic Construct
  misc_feature 7: note = locked nucleic acid
  misc_feature 12: note = locked nucleic acid
  misc_feature 14..15: note = locked nucleic acid
  source 1..18: mol_type = other DNA
atattgtaagacaatcac

SEQ ID NO: 403 - DNA, 15 bp, synthetic construct
  misc_feature 1..15: note = Synthetic Construct
  source 1..15: mol_type = other DNA
atgtggctggaccaa

SEQ ID NO: 404 - DNA, 13 bp, synthetic construct
  misc_feature 1..13: note = Synthetic Construct
  misc_feature 3: note = locked nucleic acid
  misc_feature 5: note = locked nucleic acid
  misc_feature 7: note = locked nucleic acid
  misc_feature 11: note = locked nucleic acid
  source 1..13: mol_type = other DNA
cctgaggggctgt

SEQ ID NO: 405 - DNA, 15 bp, synthetic construct
  misc_feature 1..15: note = Synthetic Construct
  source 1..15: mol_type = other DNA
ctctacgcccgacag

SEQ ID NO: 406 - DNA, 16 bp, synthetic construct
  misc_feature 1..16: note = Synthetic Construct
  misc_feature 12: note = locked nucleic acid
  source 1..16: mol_type = other DNA
ttggtggcatcatgag

SEQ ID NO: 407 - DNA, 23 bp, synthetic construct
  misc_feature 1..23: note = Synthetic Construct
  source 1..23: mol_type = other DNA
tgtcacctctgtcacaaccgagg

SEQ ID NO: 408 - DNA, 16 bp, synthetic construct
  misc_feature 1..16: note = Synthetic Construct
  source 1..16: mol_type = other DNA
acccacaccactactc

SEQ ID NO: 409 - DNA, 16 bp, synthetic construct
  misc_feature 1..16: note = Synthetic Construct
  misc_feature 16: note = locked nucleic acid
  source 1..16: mol_type = other DNA
tctggcacatgcaaga

SEQ ID NO: 410 - DNA, 26 bp, synthetic construct
  misc_feature 1..26: note = Synthetic Construct
  source 1..26: mol_type = other DNA
taccgaacttcaacccacaccatcac

SEQ ID NO: 411 - DNA, 18 bp, synthetic construct
  misc_feature 1..18: note = Synthetic Construct
  misc_feature 16: note = locked nucleic acid
  source 1..18: mol_type = other DNA
aatcaatgcaccctctta

SEQ ID NO: 412 - DNA, 20 bp, synthetic construct
  misc_feature 1..20: note = Synthetic Construct
  misc_feature 5: note = locked nucleic acid
  misc_feature 18..19: note = locked nucleic acid
  source 1..20: mol_type = other DNA
aatgttataaaatacagtcg

SEQ ID NO: 413 - DNA, 26 bp, synthetic construct
  misc_feature 1..26: note = Synthetic Construct
  source 1..26: mol_type = other DNA
tgatccagatagtccagaaccacggt

SEQ ID NO: 414 - DNA, 17 bp, synthetic construct
  misc_feature 1..17: note = Synthetic Construct
  source 1..17: mol_type = other DNA
attacccccctcacaat

SEQ ID NO: 415 - DNA, 20 bp, synthetic construct
  misc_feature 1..20: note = Synthetic Construct
  misc_feature 9: note = locked nucleic acid
  misc_feature 18: note = locked nucleic acid
  source 1..20: mol_type = other DNA
tagatgatgtaattgttggt

SEQ ID NO: 416 - DNA, 19 bp, synthetic construct
  misc_feature 1..19: note = Synthetic Construct
  source 1..19: mol_type = other DNA
caccaccagcagcaccagc

SEQ ID NO: 417 - DNA, 15 bp, synthetic construct
  misc_feature 1..15: note = Synthetic Construct
  source 1..15: mol_type = other DNA
acaagcaacgcaagc

SEQ ID NO: 418 - DNA, 18 bp, synthetic construct
  misc_feature 1..18: note = Synthetic Construct
  misc_feature 11: note = locked nucleic acid
  source 1..18: mol_type = other DNA
aggactggacttagttca

SEQ ID NO: 419 - DNA, 23 bp, synthetic construct
  misc_feature 1..23: note = Synthetic Construct
  source 1..23: mol_type = other DNA
accttggagaccagagccaaaca

SEQ ID NO: 420 - DNA, 19 bp, synthetic construct
  misc_feature 1..19: note = Synthetic Construct
  misc_feature 4: note = locked nucleic acid
  misc_feature 14: note = locked nucleic acid
  source 1..19: mol_type = other DNA
cgtttgtagaaattcacac

SEQ ID NO: 421 - DNA, 17 bp, synthetic construct
  misc_feature 1..17: note = Synthetic Construct
  misc_feature 12: note = locked nucleic acid
  source 1..17: mol_type = other DNA
tctgggctattatggga

SEQ ID NO: 422 - DNA, 14 bp, synthetic construct
  misc_feature 1..14: note = Synthetic Construct
  misc_feature 4..6: note = locked nucleic acid
  misc_feature 10..11: note = locked nucleic acid
  source 1..14: mol_type = other DNA
tcaccaatacatga

SEQ ID NO: 423 - DNA, 17 bp, synthetic construct
  misc_feature 1..17: note = Synthetic Construct
  source 1..17: mol_type = other DNA
ccattctcttccccgat

SEQ ID NO: 424 - DNA, 18 bp, synthetic construct
  misc_feature 1..18: note = Synthetic Construct
  misc_feature 9: note = locked nucleic acid
  misc_feature 15: note = locked nucleic acid
  source 1..18: mol_type = other DNA
aaatgtaatcccaacttt

SEQ ID NO: 425 - DNA, 13 bp, synthetic construct
  misc_feature 1..13: note = Synthetic Construct
  misc_feature 3..6: note = locked nucleic acid
  misc_feature 13: note = locked nucleic acid
  source 1..13: mol_type = other DNA
ccgcagacttaga